European Patent Specification EP 3 636 753 B1, published April 3, 2024. Title: METHOD FOR PRODUCING DNA-EDITED EUKARYOTIC CELL, AND KIT USED IN THE SAME. Applicant: Osaka University. The sequence listing filed with the application follows.

SEQUENCE LISTING (65 sequences)

SEQ ID NO: 1 - DNA, 2685 bp, Artificial Sequence
  modified Cas3 with NLS
atgcccaagaagaagcggaaggtggaaccttttaaatatatatgccattactggggaaaatcctcaaaaagcttgacgaaaggaaatgatattcatctgttaatttatcattgccttgatgttgctgctgttgcagattgctggtgggatcaatcagtcgtactgcaaaatactttttgccgaaatgaaatgctatcaaaacagagggtgaaggcctggctgttatttttcattgctcttcatgatattggaaagtttgatatacgattccaatataaatcagcagaaagttggctgaaattaaatcctgcaacgccatcacttaatggtccatcaacacaaatgtgccgtaaatttaatcatggtgcagccggtctgtattggtttaaccaggattcactttcagagcaatctctcggggattttttcagtttttttgatgccgctcctcatccttatgagtcctggtttccatgggtagaggccgttacaggacatcatggttttatattacattcccaggatcaagataagtcgcgttgggaaatgccagcttctctggcatcttatgctgcgcaagataaacaggctcgtgaggagtggatatctgtactggaagcattatttttaacgccagcggggttatctataaacgatataccacctgattgttcatcactgttagcaggtttttgctcgcttgctgactggttaggctcctggactacaacgaatacctttctgtttaatgaggatgcgccttccgacataaatgctctgagaacgtatttccaggaccgacagcaggatgcgagccgggtattggagttgagtggacttgtatcaaataagcgatgttatgaaggtgttcatgcactactggacaatggctatcaacccagacaattacaggtgttagttgatgctcttccagtagctcccgggctgacggtaatagaggcacctacaggctccggtaaaacggaaacagcgctggcctatgcttggaaacttattgatcaacaaattgcggatagtgttatttttgccctcccaacacaagctaccgcgaatgctatgcttacgagaatggaagcgagcgcgagccacttattttcatccccaaatcttattcttgctcatggcaattcacggtttaaccacctctttcaatcaataaaatcacgcgcgattactgaacaggggcaagaagaagcgtgggttcagtgttgtcagtggttgtcacaaagcaataagaaagtgtttcttgggcaaatcggcgtttgcacgattgatcaggtgttgatatcggtattgccagttaaacaccgctttatccgtggtttgggaattggtcgaagtgttttaattgttgatgaagttcatgcttacgacacctatatgaacggcttgctggaggcagtgctcaaggctcaggctgatgtgggagggagtgttattcttctttccgcaaccctaccaatgaaacaaaaacagaaacttctggatacttatggtctgcatacagatccagtggaaaataactccgcatatccactcattaactggcgaggtgtgaatggtgcgcaacgttttgatctgctagctcatccagaacaactcccgccccgcttttcgattcagccagaacctatttgtttagctgacatgttacctgaccttacgatgttagagcgaatgatcgcagcggcaaacgcgggtgcacaggtctgtcttatttgcaatttggttgacgttgcacaagtatgctaccaacggctaaaggagctaaataacacgcaagtagatatagatttgtttcatgcgcgctttacgctgaacgatcgtcgtgaaaaagagaatcgagttattagcaatttcggcaaaaatgggaagcgaaatgttggacggatacttgtcgcaacccaggtcgtggaacaatcactcgacgttgattttgattggttaattactcagcattgtcctgcagatttgcttttccaacgattgggccgtttacatcgccatcatcgcaaatatcgtcccgctggttttgagattcctgttgccaccattttgctgcctgatggcgagggttacggacgacatgagcatatttatagcaacgttagagtcatgtggcggacgcagcaacatattgaggagcttaatggagcatccttatttttccctgatgcttaccggcaatggctggatagcatttacgatgatgcggaaatggatgagccagaatgggtcggcaatggcatggataaatttgaaagcgccgagtgtgaaaaaaggttcaaggctcgcaaggtcctgcagtgggctgaagaatatagcttgcaggataacgatgaaaccattcttgcggtaacgagggatggggaaatgagcctgccattattgccttatgtacaaacgtcttcaggtaaacaactgctcgatggccaggtctacgaggacctaagtcatgaacagcagtatgaggcgcttgcacttaatcgcgtcaatgtacccttcacctggaaacgtagtttttctgaagtagtagatgaagatgggttactttggctggaagggaaacagaatctggatggatgggtctggcagggtaacagtattgttattacctatacaggggatgaagggatgaccagagtcatccctgcaaatcccaaa

SEQ ID NO: 2 - DNA, 1527 bp, Artificial Sequence
  modified Cse1 with NLS
atgcccaagaagaagcggaaggtgaacctgctgattgacaactggatccctgtgcgcccacggaacggaggaaaagtccagattattaatctgcagagcctgtactgctcccgggatcagtggagactgagcctgcccagagacgatatggagctggccgccctggccctgctggtgtgcatcggccagatcatcgcccctgccaaggacgatgtggagttcaggcaccgcatcatgaaccctctgaccgaggatgagtttcagcagctgatcgccccatggatcgacatgttctatctgaatcacgccgagcaccccttcatgcagacaaagggcgtgaaggccaacgacgtgacccccatggagaagctgctggcaggcgtgtccggagcaacaaattgcgccttcgtgaaccagccaggacagggagaggccctgtgcggaggctgtaccgccatcgccctgtttaatcaggcaaaccaggcacctggattcggaggaggctttaagtctggactgaggggaggaaccccagtgaccacattcgtgagaggcatcgatctgaggagcacagtgctgctgaatgtgctgaccctgccacggctgcagaagcagtttcccaatgagagccacacagagaaccagcccacctggatcaagcctatcaagtctaacgagagcatccctgccagctccatcggcttcgtgagaggcctgttttggcagccagcccacatcgagctgtgcgaccccatcggcatcggcaagtgttcttgctgtggccaggaaagcaatctgaggtacaccggcttcctgaaggagaagttcacctttacagtgaacggcctgtggccccaccctcactctccatgtctggtgacagtgaagaagggcgaggtggaggagaagttcctggcctttaccacatccgccccctcttggacccagatcagcagagtggtggtggacaagatcatccagaacgagaatggcaacagagtggccgccgtggtgaatcagttcaggaacatcgccccacagtctcccctggagctgatcatgggcggctacaggaacaatcaggccagcatcctggagcggagacacgatgtgctgatgtttaatcagggctggcagcagtatggcaatgtgatcaacgagatcgtgacagtgggcctgggctacaagaccgccctgagaaaggccctgtatacattcgccgagggctttaagaacaaggacttcaagggagcaggcgtgagcgtgcacgagaccgccgagaggcacttttaccgccagtccgagctgctgatccccgatgtgctggccaatgtgaacttctcccaggccgacgaagtgatcgccgatctgagggacaagctgcaccagctgtgcgagatgctgtttaaccagtctgtggccccatacgcccaccaccccaagctgatcagcacactggccctggcaagggccaccctgtataagcacctgagggagctgaagccacagggaggaccttctaatgga

SEQ ID NO: 3 - DNA, 501 bp, Artificial Sequence
  modified Cse2 with NLS
atgcccaagaagaagcggaaggtggccgatgagatcgacgcaatggcactgtacagggcatggcagcagctggacaacggatcttgcgcacagatcaggcgcgtgagcgagcctgatgagctgagggacatcccagccttctatcggctggtgcagccctttggctgggagaatcctagacaccagcaggccctgctgaggatggtgttttgtctgagcgccggcaagaacgtgatccggcaccaggacaagaagagcgagcagaccacaggaatctccctgggacgcgccctggccaattccggccggatcaacgagcggagaatcttccagctgatcagggccgatcgcacagccgacatggtgcagctgaggcgcctgctgacccacgcagagcctgtgctggattggccactgatggcccgcatgctgacatggtggggcaagcgggagagacagcagctgctggaggacttcgtgctgaccacaaataagaacgcc

SEQ ID NO: 4 - DNA, 693 bp, Artificial Sequence
  modified Cas5 with NLS
atgcccaagaagaagcggaaggtgcgctcctacctgatcctgagactggcaggaccaatgcaggcatggggacagcctacattcgagggaaccaggccaacaggccgctttcctacccggtctggactgctgggactgctgggagcctgcctgggcatccagagggacgatacctctagcctgcaggccctgagcgagtccgtgcagttcgccgtgcgctgtgatgagctgatcctggacgataggcgcgtgtccgtgacaggcctgcgggattaccacaccgtgctgggcgccagagaggactataggggcctgaagtcccacgagaccatccagacatggcgcgagtacctgtgcgacgcctcttttacagtggccctgtggctgaccccacacgcaacaatggtcatcagcgagctggagaaggccgtgctgaagccacggtacaccccctatctgggccggagaagctgccctctgacacacccactgttcctgggcacctgtcaggcctccgatccccagaaggccctgctgaactacgagcctgtgggcggcgacatctattctgaggagagcgtgacaggccaccacctgaagttcaccgccagggatgagccaatgatcacactgccaaggcagtttgcatccagggagtggtatgtgatcaagggaggaatggacgtgagccag

SEQ ID NO: 5 - DNA, 618 bp, Artificial Sequence
  modified Cas6 with NLS
atgcccaagaagaagcggaaggtgtacctgagcaaagtgatcatcgcaagggcatggtccagggacctgtatcagctgcaccagggcctgtggcacctgttccctaatagaccagatgccgccagggacttcctgtttcacgtggagaagaggaacacacccgagggctgtcacgtgctgctgcagtccgcccagatgcccgtgagcaccgcagtggccacagtgatcaagaccaagcaggtggagttccagctgcaagtgggcgtgccactgtactttaggctgcgcgccaatcccatcaagaccatcctggataaccagaagcgcctggactctaagggcaatatcaagcggtgcagagtgcctctgatcaaggaggccgagcagatcgcctggctgcagagaaagctgggcaacgccgccagggtggaggatgtgcaccctatcagcgagcggccacagtatttcagcggcgacggcaagtccggcaagatccagaccgtgtgctttgagggcgtgctgaccatcaacgatgccccagccctgatcgacctggtgcagcagggaatcggacctgctaagtcaatgggatgtgggctgctgtcactggcacctctg

SEQ ID NO: 6 - DNA, 1110 bp, Artificial Sequence
  modified Cas7 with NLS
atgcccaagaagaagcggaaggtgtccaatttcatcaacatccacgtgctgatctcccactctccaagctgcctgaatagagacgatatgaacatgcagaaggacgccatctttggcggcaagcggagagtgaggatctctagccagtccctgaagcgggccatgagaaagtctggctactatgcccagaatatcggcgagtcctctctgaggaccatccacctggcacagctgagggacgtgctgagacagaagctgggcgagcggtttgatcagaagatcatcgacaagacactggccctgctgagcggcaagtccgtggatgaggccgagaagatcagcgccgacgcagtgaccccatgggtggtgggagagatcgcatggttctgtgagcaggtggccaaggccgaggccgataatctggacgataagaagctgctgaaggtgctgaaggaggatatcgccgccatcagagtgaacctgcagcagggagtggacatcgccctgagcggcaggatggccacatccggcatgatgaccgagctgggcaaggtggacggagcaatgtccatcgcacacgccatcaccacacaccaggtggactctgatatcgactggttcacagccgtggacgatctgcaggagcagggaagcgcccacctgggaacccaggagttcagctccggcgtgttttacagatatgccaatatcaacctggcacagctgcaggagaacctgggaggagcatccagggagcaggccctggagatcgccacacacgtggtgcacatgctggcaaccgaggtgccaggagcaaagcagcgcacctacgccgccttcaatcctgccgatatggtcatggtgaacttttccgacatgccactgtctatggccaatgccttcgagaaggccgtgaaggccaaggatggcttcctgcagccttccatccaggcctttaaccagtactgggaccgcgtggccaatggatatggcctgaacggagctgccgcccagttttccctgtctgatgtggaccctatcacagcccaggtgaagcagatgccaaccctggagcagctgaagagctgggtgcggaacaatggagaggca

SEQ ID NO: 7 - DNA, 2775 bp, Artificial Sequence
  modified Cas3 with BPNLS
aagcggactgctgatggcagtgaatttgagtccccaaagaagaagagaaaggtggaagaaccttttaaatatatatgccattactggggaaaatcctcaaaaagcttgacgaaaggaaatgatattcatctgttaatttatcattgccttgatgttgctgctgttgcagattgctggtgggatcaatcagtcgtactgcaaaatactttttgccgaaatgaaatgctatcaaaacagagggtgaaggcctggctgttatttttcattgctcttcatgatattggaaagtttgatatacgattccaatataaatcagcagaaagttggctgaaattaaatcctgcaacgccatcacttaatggtccatcaacacaaatgtgccgtaaatttaatcatggtgcagccggtctgtattggtttaaccaggattcactttcagagcaatctctcggggattttttcagtttttttgatgccgctcctcatccttatgagtcctggtttccatgggtagaggccgttacaggacatcatggttttatattacattcccaggatcaagataagtcgcgttgggaaatgccagcttctctggcatcttatgctgcgcaagataaacaggctcgtgaggagtggatatctgtactggaagcattatttttaacgccagcggggttatctataaacgatataccacctgattgttcatcactgttagcaggtttttgctcgcttgctgactggttaggctcctggactacaacgaatacctttctgtttaatgaggatgcgccttccgacataaatgctctgagaacgtatttccaggaccgacagcaggatgcgagccgggtattggagttgagtggacttgtatcaaataagcgatgttatgaaggtgttcatgcactactggacaatggctatcaacccagacaattacaggtgttagttgatgctcttccagtagctcccgggctgacggtaatagaggcacctacaggctccggtaaaacggaaacagcgctggcctatgcttggaaacttattgatcaacaaattgcggatagtgttatttttgccctcccaacacaagctaccgcgaatgctatgcttacgagaatggaagcgagcgcgagccacttattttcatccccaaatcttattcttgctcatggcaattcacggtttaaccacctctttcaatcaataaaatcacgcgcgattactgaacaggggcaagaagaagcgtgggttcagtgttgtcagtggttgtcacaaagcaataagaaagtgtttcttgggcaaatcggcgtttgcacgattgatcaggtgttgatatcggtattgccagttaaacaccgctttatccgtggtttgggaattggtcgaagtgttttaattgttgatgaagttcatgcttacgacacctatatgaacggcttgctggaggcagtgctcaaggctcaggctgatgtgggagggagtgttattcttctttccgcaaccctaccaatgaaacaaaaacagaaacttctggatacttatggtctgcatacagatccagtggaaaataactccgcatatccactcattaactggcgaggtgtgaatggtgcgcaacgttttgatctgctagctcatccagaacaactcccgccccgcttttcgattcagccagaacctatttgtttagctgacatgttacctgaccttacgatgttagagcgaatgatcgcagcggcaaacgcgggtgcacaggtctgtcttatttgcaatttggttgacgttgcacaagtatgctaccaacggctaaaggagctaaataacacgcaagtagatatagatttgtttcatgcgcgctttacgctgaacgatcgtcgtgaaaaagagaatcgagttattagcaatttcggcaaaaatgggaagcgaaatgttggacggatacttgtcgcaacccaggtcgtggaacaatcactcgacgttgattttgattggttaattactcagcattgtcctgcagatttgcttttccaacgattgggccgtttacatcgccatcatcgcaaatatcgtcccgctggttttgagattcctgttgccaccattttgctgcctgatggcgagggttacggacgacatgagcatatttatagcaacgttagagtcatgtggcggacgcagcaacatattgaggagcttaatggagcatccttatttttccctgatgcttaccggcaatggctggatagcatttacgatgatgcggaaatggatgagccagaatgggtcggcaatggcatggataaatttgaaagcgccgagtgtgaaaaaaggttcaaggctcgcaaggtcctgcagtgggctgaagaatatagcttgcaggataacgatgaaaccattcttgcggtaacgagggatggggaaatgagcctgccattattgccttatgtacaaacgtcttcaggtaaacaactgctcgatggccaggtctacgaggacctaagtcatgaacagcagtatgaggcgcttgcacttaatcgcgtcaatgtacccttcacctggaaacgtagtttttctgaagtagtagatgaagatgggttactttggctggaagggaaacagaatctggatggatgggtctggcagggtaacagtattgttattacctatacaggggatgaagggatgaccagagtcatccctgcaaatcccaaaaagcggactgctgatggcagtgaatttgagtccccaaagaagaagagaaaggtggaa

SEQ ID NO: 8 - DNA, 1617 bp, Artificial Sequence
  modified Cse1 with BPNLS
aagcggactgctgatggcagtgaatttgagtccccaaagaagaagagaaaggtggaaaacctgctgattgacaactggatccctgtgcgcccacggaacggaggaaaagtccagattattaatctgcagagcctgtactgctcccgggatcagtggagactgagcctgcccagagacgatatggagctggccgccctggccctgctggtgtgcatcggccagatcatcgcccctgccaaggacgatgtggagttcaggcaccgcatcatgaaccctctgaccgaggatgagtttcagcagctgatcgccccatggatcgacatgttctatctgaatcacgccgagcaccccttcatgcagacaaagggcgtgaaggccaacgacgtgacccccatggagaagctgctggcaggcgtgtccggagcaacaaattgcgccttcgtgaaccagccaggacagggagaggccctgtgcggaggctgtaccgccatcgccctgtttaatcaggcaaaccaggcacctggattcggaggaggctttaagtctggactgaggggaggaaccccagtgaccacattcgtgagaggcatcgatctgaggagcacagtgctgctgaatgtgctgaccctgccacggctgcagaagcagtttcccaatgagagccacacagagaaccagcccacctggatcaagcctatcaagtctaacgagagcatccctgccagctccatcggcttcgtgagaggcctgttttggcagccagcccacatcgagctgtgcgaccccatcggcatcggcaagtgttcttgctgtggccaggaaagcaatctgaggtacaccggcttcctgaaggagaagttcacctttacagtgaacggcctgtggccccaccctcactctccatgtctggtgacagtgaagaagggcgaggtggaggagaagttcctggcctttaccacatccgccccctcttggacccagatcagcagagtggtggtggacaagatcatccagaacgagaatggcaacagagtggccgccgtggtgaatcagttcaggaacatcgccccacagtctcccctggagctgatcatgggcggctacaggaacaatcaggccagcatcctggagcggagacacgatgtgctgatgtttaatcagggctggcagcagtatggcaatgtgatcaacgagatcgtgacagtgggcctgggctacaagaccgccctgagaaaggccctgtatacattcgccgagggctttaagaacaaggacttcaagggagcaggcgtgagcgtgcacgagaccgccgagaggcacttttaccgccagtccgagctgctgatccccgatgtgctggccaatgtgaacttctcccaggccgacgaagtgatcgccgatctgagggacaagctgcaccagctgtgcgagatgctgtttaaccagtctgtggccccatacgcccaccaccccaagctgatcagcacactggccctggcaagggccaccctgtataagcacctgagggagctgaagccacagggaggaccttctaatggaaagcggactgctgatggcagtgaatttgagtccccaaagaagaagagaaaggtggaa

SEQ ID NO: 9 - DNA, 591 bp, Artificial Sequence
  modified Cse2 with BPNLS
aagcggactgctgatggcagtgaatttgagtccccaaagaagaagagaaaggtggaagccgatgagatcgacgcaatggcactgtacagggcatggcagcagctggacaacggatcttgcgcacagatcaggcgcgtgagcgagcctgatgagctgagggacatcccagccttctatcggctggtgcagccctttggctgggagaatcctagacaccagcaggccctgctgaggatggtgttttgtctgagcgccggcaagaacgtgatccggcaccaggacaagaagagcgagcagaccacaggaatctccctgggacgcgccctggccaattccggccggatcaacgagcggagaatcttccagctgatcagggccgatcgcacagccgacatggtgcagctgaggcgcctgctgacccacgcagagcctgtgctggattggccactgatggcccgcatgctgacatggtggggcaagcgggagagacagcagctgctggaggacttcgtgctgaccacaaataagaacgccaagcggactgctgatggcagtgaatttgagtccccaaagaagaagagaaaggtggaa

SEQ ID NO: 10 - DNA, 783 bp, Artificial Sequence
  modified Cas5 with BPNLS
aagcggactgctgatggcagtgaatttgagtccccaaagaagaagagaaaggtggaacgctcctacctgatcctgagactggcaggaccaatgcaggcatggggacagcctacattcgagggaaccaggccaacaggccgctttcctacccggtctggactgctgggactgctgggagcctgcctgggcatccagagggacgatacctctagcctgcaggccctgagcgagtccgtgcagttcgccgtgcgctgtgatgagctgatcctggacgataggcgcgtgtccgtgacaggcctgcgggattaccacaccgtgctgggcgccagagaggactataggggcctgaagtcccacgagaccatccagacatggcgcgagtacctgtgcgacgcctcttttacagtggccctgtggctgaccccacacgcaacaatggtcatcagcgagctggagaaggccgtgctgaagccacggtacaccccctatctgggccggagaagctgccctctgacacacccactgttcctgggcacctgtcaggcctccgatccccagaaggccctgctgaactacgagcctgtgggcggcgacatctattctgaggagagcgtgacaggccaccacctgaagttcaccgccagggatgagccaatgatcacactgccaaggcagtttgcatccagggagtggtatgtgatcaagggaggaatggacgtgagccagaagcggactgctgatggcagtgaatttgagtccccaaagaagaagagaaaggtggaa

SEQ ID NO: 11 - DNA, 708 bp, Artificial Sequence
  modified Cas6 with BPNLS
aagcggactgctgatggcagtgaatttgagtccccaaagaagaagagaaaggtggaatacctgagcaaagtgatcatcgcaagggcatggtccagggacctgtatcagctgcaccagggcctgtggcacctgttccctaatagaccagatgccgccagggacttcctgtttcacgtggagaagaggaacacacccgagggctgtcacgtgctgctgcagtccgcccagatgcccgtgagcaccgcagtggccacagtgatcaagaccaagcaggtggagttccagctgcaagtgggcgtgccactgtactttaggctgcgcgccaatcccatcaagaccatcctggataaccagaagcgcctggactctaagggcaatatcaagcggtgcagagtgcctctgatcaaggaggccgagcagatcgcctggctgcagagaaagctgggcaacgccgccagggtggaggatgtgcaccctatcagcgagcggccacagtatttcagcggcgacggcaagtccggcaagatccagaccgtgtgctttgagggcgtgctgaccatcaacgatgccccagccctgatcgacctggtgcagcagggaatcggacctgctaagtcaatgggatgtgggctgctgtcactggcacctctgaagcggactgctgatggcagtgaatttgagtccccaaagaagaagagaaaggtggaa

SEQ ID NO: 12 - DNA, 1200 bp, Artificial Sequence
  modified Cas7 with BPNLS
aagcggactgctgatggcagtgaatttgagtccccaaagaagaagagaaaggtggaatccaatttcatcaacatccacgtgctgatctcccactctccaagctgcctgaatagagacgatatgaacatgcagaaggacgccatctttggcggcaagcggagagtgaggatctctagccagtccctgaagcgggccatgagaaagtctggctactatgcccagaatatcggcgagtcctctctgaggaccatccacctggcacagctgagggacgtgctgagacagaagctgggcgagcggtttgatcagaagatcatcgacaagacactggccctgctgagcggcaagtccgtggatgaggccgagaagatcagcgccgacgcagtgaccccatgggtggtgggagagatcgcatggttctgtgagcaggtggccaaggccgaggccgataatctggacgataagaagctgctgaaggtgctgaaggaggatatcgccgccatcagagtgaacctgcagcagggagtggacatcgccctgagcggcaggatggccacatccggcatgatgaccgagctgggcaaggtggacggagcaatgtccatcgcacacgccatcaccacacaccaggtggactctgatatcgactggttcacagccgtggacgatctgcaggagcagggaagcgcccacctgggaacccaggagttcagctccggcgtgttttacagatatgccaatatcaacctggcacagctgcaggagaacctgggaggagcatccagggagcaggccctggagatcgccacacacgtggtgcacatgctggcaaccgaggtgccaggagcaaagcagcgcacctacgccgccttcaatcctgccgatatggtcatggtgaacttttccgacatgccactgtctatggccaatgccttcgagaaggccgtgaaggccaaggatggcttcctgcagccttccatccaggcctttaaccagtactgggaccgcgtggccaatggatatggcctgaacggagctgccgcccagttttccctgtctgatgtggaccctatcacagcccaggtgaagcagatgccaaccctggagcagctgaagagctgggtgcggaacaatggagaggcaaagcggactgctgatggcagtgaatttgagtccccaaagaagaagagaaaggtggaa

SEQ ID NO: 13 - DNA, 2664 bp, Escherichia coli
atggagccattcaaatacatctgccactactgggggaaatcatctaaaagcctgacaaaggggaacgatatccacctgctgatctaccactgcctggacgtggcagcagtggcagattgttggtgggaccagagcgtggtgctgcagaataccttctgccggaacgagatgctgtccaagcagagagtgaaggcctggctgctgttctttatcgccctgcacgatatcggcaagttcgacatcaggtttcagtataagtctgccgagagctggctgaagctgaatccagccacaccctccctgaacggcccttctacccagatgtgcaggaagttcaatcacggagcagcaggactgtactggtttaaccaggacagcctgtccgagcagtctctgggcgatttctttagcttctttgacgccgcccctcacccatatgagagctggttcccatgggtggaggcagtgacaggacaccacggctttatcctgcactcccaggaccaggataagtctagatgggagatgccagcatccctggcatcttacgcagcacaggataagcaggcaagggaggagtggatctctgtgctggaggccctgttcctgaccccagcaggcctgagcatcaatgatatcccacctgactgcagctccctgctggcaggcttttgtagcctggcagactggctgggatcctggaccacaaccaatacattcctgtttaacgaggatgccccttctgacatcaacgccctgcgcacctacttccaggatcggcagcaggacgccagcagagtgctggagctgtctggcctggtgagcaataagcggtgctacgagggagtgcacgcactgctggataacggctatcagcctagacagctgcaggtgctggtggacgcactgcctgtggcaccaggactgacagtgatcgaggcaccaaccggctctggcaagacagagaccgccctggcctatgcctggaagctgatcgatcagcagatcgccgacagcgtgatcttcgcactgccaacacaggcaaccgcaaatgccatgctgaccaggatggaggcctctgccagccacctgttttctagccctaacctgatcctggcccacggcaacagccggttcaatcacctgtttcagagcatcaagtccagagccatcacagagcagggacaggaggaggcatgggtgcagtgctgtcagtggctgtcccagtctaacaagaaggtgttcctgggccagatcggcgtgtgcaccatcgatcaggtgctgatctccgtgctgccagtgaagcacaggtttatcaggggactgggaatcggccgctctgtgctgatcgtggatgaggtgcacgcctacgacacatatatgaacggcctgctggaggccgtgctgaaggcacaggcagacgtgggaggaagcgtgatcctgctgtccgccaccctgcccatgaagcagaagcagaagctgctggatacatacggcctgcacaccgaccctgtggagaacaatagcgcctatccactgatcaattggaggggagtgaacggagcacagcggttcgacctgctggcacacccagagcagctgccaccacggttttccatccagcccgagcctatctgcctggccgatatgctgcccgacctgaccatgctggagagaatgatcgctgccgccaatgcaggagcacaggtgtgcctgatctgtaacctggtggatgtggcccaggtgtgctaccagcggctgaaggagctgaacaatacacaggtggacatcgatctgttccacgccaggtttaccctgaatgaccggagagagaaggagaaccgcgtgatctccaacttcggcaagaatggcaagagaaacgtgggcaggatcctggtggccacacaggtggtggagcagtctctggacgtggatttcgactggctgatcacccagcactgccctgccgatctgctgtttcagcggctgggcagactgcacagacaccacaggaagtacaggccagcaggatttgagatcccagtggccacaatcctgctgccagacggagagggatacggccggcacgagcacatctatagcaatgtgcgcgtgatgtggcggacccagcagcacatcgaggagctgaacggcgcctccctgttctttcccgatgcctacagacagtggctggactctatctatgacgatgccgagatggatgagcctgagtgggtgggcaatggcatggacaagttcgagtccgccgagtgtgagaagcggttcaaggccaggaaggtgctgcagtgggccgaggagtacagcctgcaggataacgacgagacaatcctggccgtgaccagggatggcgagatgtccctgcccctgctgccttatgtgcagacatcctctggcaagcagctgctggatggccaggtgtacgaggacctgagccacgagcagcagtatgaggccctggccctgaacagggtgaatgtgcccttcacctggaagcgcagcttttccgaagtggtggatgaggacggcctgctgtggctggagggcaagcagaatctggacggctgggtgtggcagggcaactccatcgtgattacctacaccggagacgaagggatgacaagagtgattcctgctaacccaaag

SEQ ID NO: 14 - DNA, 1506 bp, Escherichia coli
atgaatttgcttattgataactggatccctgtacgcccgcgaaacggggggaaagtccaaatcataaatctgcaatcgctatactgcagtagagatcagtggcgattaagtttgccccgtgacgatatggaactggccgctttagcactgctggtttgcattgggcaaattatcgccccggcaaaagatgacgttgaatttcgacatcgcataatgaatccgctcactgaagatgagtttcaacaactcatcgcgccgtggatagatatgttctaccttaatcacgcagaacatccctttatgcagaccaaaggtgtcaaagcaaatgatgtgactccaatggaaaaactgttggctggggtaagcggcgcgacgaattgtgcatttgtcaatcaaccggggcagggtgaagcattatgtggtggatgcactgcgattgcgttattcaaccaggcgaatcaggcaccaggttttggtggtggttttaaaagcggtttacgtggaggaacacctgtaacaacgttcgtacgtgggatcgatcttcgttcaacggtgttactcaatgtcctcacattacctcgtcttcaaaaacaatttcctaatgaatcacatacggaaaaccaacctacctggattaaacctatcaagtccaatgagtctatacctgcttcgtcaattgggtttgtccgtggtctattctggcaaccagcgcatattgaattatgcgatcccattgggattggtaaatgttcttgctgtggacaggaaagcaatttgcgttataccggttttcttaaggaaaaatttacctttacagttaatgggctatggccccatccgcattccccttgtctggtaacagtcaagaaaggggaggttgaggaaaaatttcttgctttcaccacctccgcaccatcatggacacaaatcagccgagttgtggtagataagattattcaaaatgaaaatggaaatcgcgtggcggcggttgtgaatcaattcagaaatattgcgccgcaaagtcctcttgaattgattatggggggatatcgtaataatcaagcatctattcttgaacggcgtcatgatgtgttgatgtttaatcaggggtggcaacaatacggcaatgtgataaacgaaatagtgactgttggtttgggatataaaacagccttacgcaaggcgttatatacctttgcagaagggtttaaaaataaagacttcaaaggggccggagtctctgttcatgagactgcagaaaggcatttctatcgacagagtgaattattaattcccgatgtactggcgaatgttaatttttcccaggctgatgaggtaatagctgatttacgagacaaacttcatcaattgtgtgaaatgctatttaatcaatctgtagctccctatgcacatcatcctaaattaataagcacattagcgcttgcccgcgccacgctatacaaacatttacgggagttaaaaccgcaaggagggccatcaaatggc

SEQ ID NO: 15 - DNA, 480 bp, Escherichia coli
atggctgatgaaattgatgcaatggctttatatcgagcctggcaacaactggataatggatcatgtgcgcaaattagacgtgtttcagaacctgatgaattacgcgatatccctgcgttttataggctggtgcaaccttttggttgggaaaacccacgtcaccagcaggctcttttgcgcatggtgttttgcctgagcgcaggaaagaatgtcatccgacatcaggacaaaaaatcggagcaaacaacaggtatctcgttgggaagagctttagccaatagtggaagaattaacgagcgccgtatctttcaattaattcgggctgacagaacagccgatatggtccagttacgtcgattacttactcacgccgaacccgtacttgactggccattaatggccaggatgttgacctggtggggaaagcgcgaacgccagcaacttctggaagattttgtattgaccacaaacaaaaatgcg

SEQ ID NO: 16 - DNA, 672 bp, Escherichia coli
atgagatcttatttgatcttgcggcttgctgggccaatgcaagcctgggggcagccgacctttgaaggaacgcgacctaccggaagatttccgacccgaagcgggttattagggctactcggggcttgtcttgggatccaacgtgatgatacttcttcattacaggcgttatcagagagtgtgcaatttgcagtgcgctgcgatgaactcattcttgacgatcgtcgtgtgtctgtaacggggttgcgtgattaccatacagtccttggagcgcgagaagattaccgtggtttgaaaagtcatgaaacgattcaaacatggcgcgaatatttatgtgatgcctcctttaccgtcgctctctggttaacaccccatgcaacgatggttatctcagaacttgaaaaagcagtattaaagcctcggtatacaccttacctggggcggagaagttgcccactaacacacccgctttttttggggacatgtcaggcatcggatcctcagaaggcgctattaaattatgagcccgttggcggcgatatatatagtgaggaatcagttacagggcatcatttaaaatttacggcgcgcgacgaaccgatgatcaccttgcctcgacaatttgcttcccgagaatggtatgtgattaaaggaggtatggatgtatctcag

SEQ ID NO: 17 - DNA, 597 bp, Escherichia coli
atgtatctcagtaaagtcatcattgccagggcctggagcagggatctttaccaacttcaccagggattatggcatttatttccaaacagaccggatgctgctcgtgattttctttttcatgttgagaagcgaaacacaccagaaggctgtcatgttttattgcagtcagcgcaaatgcctgtttcaactgccgttgcgacagtcattaaaactaaacaggttgaatttcaacttcaggttggtgttccactctattttcggcttcgggcaaatccgatcaaaactattctcgacaatcaaaagcgcctggacagtaaagggaatattaaacgctgtcgggttccgttaataaaagaagcagaacaaatcgcgtggttgcaacgtaaattgggcaatgcggcgcgcgttgaagatgtgcatcccatatcggaacggccacagtatttttctggtgatggtaaaagtggaaagatccaaacggtttgctttgaaggtgtgctcaccatcaacgacgcgccagcgttaatagatcttgtacagcaaggtattgggccagctaaatcgatgggatgtggcttgctatctttggctccactg

SEQ ID NO: 18 - DNA, 1086 bp, Escherichia coli
tctaactttatcaatattcatgttctgatctctcacagcccttcatgtctgaaccgcgacgatatgaacatgcagaaagacgctattttcggcggcaaaagacgagtaagaatttcaagtcaaagccttaaacgtgcgatgcgtaaaagtggttattacgcacaaaatattggtgaatccagtctcagaaccattcatcttgcacaattacgtgatgttcttcggcaaaaacttggtgaacgttttgaccaaaaaatcatcgataagacattagcgctgctctccggtaaatcagttgatgaagccgaaaagatttctgccgatgcggttactccctgggttgtgggagaaatagcctggttctgtgagcaggttgcaaaagcagaggctgataatctggatgataaaaagctgctcaaagttcttaaggaagatattgccgccatacgtgtgaatttacagcagggtgttgatattgcgcttagtggaagaatggcaaccagcggcatgatgactgagttgggaaaagttgatggtgcaatgtccattgcgcatgcgatcactactcatcaggttgattctgatattgactggttcaccgctgtagatgatttacaggaacaaggttctgcacatctgggaactcaggaattttcatcgggtgttttttatcgttatgccaacattaacctcgctcaacttcaggaaaatttaggtggtgcctccagggagcaggctctggaaattgcaacccatgttgttcatatgctggcaacagaggtccctggagcaaaacagcgtacttatgccgcttttaaccctgcggatatggtaatggttaatttctccgatatgccactttctatggcaaatgcttttgaaaaagcggttaaagcgaaagatggctttttgcaaccgtctatacaggcgtttaatcaatattgggatcgcgttgccaatggatatggtctgaacggagctgctgcgcaattcagcttatctgatgtagacccaattactgctcaagttaaacaaatgcctactttagaacagttaaaatcctgggttcgtaataatggcgaggcg

SEQ ID NO: 19 - DNA, 39 bp, Artificial Sequence
  target (CCR5)
tcaagtccaatctatgacatcaattattatacatcggag

SEQ ID NO: 20 - DNA, 50 bp, Artificial Sequence
  reporter vector insert1 (CCR5)
gtcggattcaagtccaatctatgacatcaattattatacatcggagaggt

SEQ ID NO: 21 - DNA, 50 bp, Artificial Sequence
  reporter vector insert2 (CCR5)
cggtacctctccgatgtataataattgatgtcatagattggacttgaatc

SEQ ID NO: 22 - DNA, 35 bp, Artificial Sequence
  target (E. coli)
aagagcacaaatatcatcgctcaaaccacttacgg

SEQ ID NO: 23 - DNA, 46 bp, Artificial Sequence
  reporter vector insert1 (E. coli)
gtcggataagagcacaaatatcatcgctcaaaccacttacggaggt

SEQ ID NO: 24 - DNA, 46 bp, Artificial Sequence
  reporter vector insert2 (E. coli)
cggtacctccgtaagtggtttgagcgatgatatttgtgctcttatc

SEQ ID NO: 25 - DNA, 36 bp, Artificial Sequence
  crRNA insert1 (CCR5)
accgtccaatctatgacatcaattattatacatcgg

SEQ ID NO: 26 - DNA, 36 bp, Artificial Sequence
  crRNA insert 2(CCR5)
acacccgatgtataataattgatgtcatagattgga

SEQ ID NO: 27 - DNA, 36 bp, Artificial Sequence
  crRNA insert1 (E.coli)
accgagcacaaatatcatcgctcaaaccacttacgg

SEQ ID NO: 28 - DNA, 36 bp, Artificial Sequence
  crRNA insert 2(E.coli)
acacccgtaagtggtttgagcgatgatatttgtgct

SEQ ID NO: 29 - DNA, 36 bp, Artificial Sequence
  crRNA insert 1(EMX1)
accgcaggccaatggggaggacatcgatgtcacctc

SEQ ID NO: 30 - DNA, 36 bp, Artificial Sequence
  crRNA insert 2(EMX1)
acacgaggtgacatcgatgtcctccccattggcctg

SEQ ID NO: 31 - DNA, 5701 bp, Artificial Sequence
  reporter vector (CCR5)
ggcctaactggccggtacctagttattaatagtaatcaattacggggtcattagttcatagcccatatatggagttccgcgttacataacttacggtaaatggcccgcctggctgaccgcccaacgacccccgcccattgacgtcaataatgacgtatgttcccatagtaacgccaatagggactttccattgacgtcaatgggtggagtatttacggtaaactgcccacttggcagtacatcaagtgtatcatatgccaagtacgccccctattgacgtcaatgacggtaaatggcccgcctggcattatgcccagtacatgaccttatgggactttcctacttggcagtacatctacgtattagtcatcgctattaccatggtgatgcggttttggcagtacatcaatgggcgtggatagcggtttgactcacggggatttccaagtctccaccccattgacgtcaatgggagtttgttttggcaccaaaatcaacgggactttccaaaatgtcgtaacaactccgccccattgacgcaaatgggcggtaggcgtgtacggtgggaggtctatataagcagagctggtttagtgaaccgtcagatccgctagcgctaccggactcagatctcgagctcaagcttggcaatccggtactgttggtaaagccaccatggaagatgccaaaaacattaagaagggcccagcgccattctacccactcgaagacgggaccgccggcgagcagctgcacaaagccatgaagcgctacgccctggtgcccggcaccatcgcctttaccgacgcacatatcgaggtggacattacctacgccgagtacttcgagatgagcgttcggctggcagaagctatgaagcgctatgggctgaatacaaaccatcggatcgtggtgtgcagcgagaatagcttgcagttcttcatgcccgtgttgggtgccctgttcatcggtgtggctgtggccccagctaacgacatctacaacgagcgcgagctgctgaacagcatgggcatcagccagcccaccgtcgtattcgtgagcaagaaagggctgcaaaagatcctcaacgtgcaaaagaagctaccgatcatacaaaagatcatcatcatggatagcaagaccgactaccagggcttccaaagcatgtacaccttcgtgacttcccatttgccacccggcttcaacgagtacgacttcgtgcccgagagcttcgaccgggacaaaaccatcgccctgatcatgaacagtagtggcagtaccggattgcccaagggcgtagccctaccgcaccgcaccgcttgtgtccgattcagtcatgcccgcgaccccatcttcggcaaccagatcatccccgacaccgctatcctcagcgtggtgccatttcaccacggcttcggcatgttcaccacgctgggctacttgatctgcggctttcgggtcgtgctcatgtaccgcttcgaggaggagctattcttgcgcagcttgcaagactataagattcaatctgccctgctggtgcccacactatttagcttcttcgctaagagcactctcatcgacaagtacgacctaagcaacttgcacgagatcgccagcggcggggcgccgctcagcaaggaggtaggtgaggccgtggccaaacgcttccacctaccaggcatccgccagggctacggcctgacagaaacaaccagcgccattctgatcacccccgaaggggacgacaagcctggcgcagtaggcaaggtggtgcccttcttcgaggctaaggtggtggacttggactagggtctctgtcggattcaagtccaatctatgacatcaattattatacatcggagaggtaccgtgagacctaggagcgcgagctgctgaacagcatgggcatcagccagcccaccgtcgtattcgtgagcaagaaagggctgcaaaagatcctcaacgtgcaaaagaagctaccgatcatacaaaagatcatcatcatggatagcaagaccgactaccagggcttccaaagcatgtacaccttcgtgacttcccatttgccacccggcttcaacgagtacgacttcgtgcccgagagcttcgaccgggacaaaaccatcgccctgatcatgaacagtagtggcagtaccggattgcccaagggcgtagccctaccgcaccgcaccgcttgtgtccgattcagtcatgcccgcgaccccatcttcggcaaccagatcatccccgacaccgctatcctcagcgtggtgccatttcaccacggcttcggcatgttcaccacgctgggctacttgatctgcggctttcgggtcgtgctcatgtaccgcttcgaggaggagctattcttgcgcagcttgcaagactataagattcaatctgccctgctggtgcccacactatttagcttcttcgctaagagcactctcatcgacaagtacgacctaagcaacttgcacgagatcgccagcggcggggcgccgctcagcaaggaggtaggtgaggccgtggccaaacgcttccacctaccaggcatccgccagggctacggcctgacagaaacaaccagcgccattctgatcacccccgaaggggacgacaagcctggcgcagtaggcaaggtggtgcccttcttcgaggctaaggtggtggacttggacaccggtaagacactgggtgtgaaccagcgcggcgagctgtgcgtccgtggccccatgatcatgagcggctacgttaacaaccccgaggctacaaacgctctcatcgacaaggacggctggctgcacagcggcgacatcgcctactgggacgaggacgagcacttcttcatcgtggaccggctgaagagcctgatcaaatacaagggctaccaggtagccccagccgaactggagagcatcctgctgcaacaccccaacatcttcgacgccggggtcgccggcctgcccgacgacgatgccggcgagctgcccgccgcagtcgtcgtgctggaacacggtaaaaccatgaccgagaaggagatcgtggactatgtggccagccaggttacaaccgccaagaagctgcgcggtggtgttgtgttcgtggacgaggtgcctaaaggactgaccggcaagttggacgcccgcaagatccgcgagattctcattaaggccaagaagggcggcaagatcgccgtgaattcttaactgcagtctagagtcggggcggccggccgcttcgagcagacatgataagatacattgatgagtttggacaaaccacaactagaatgcagtgaaaaaaatgctttatttgtgaaatttgtgatgctattgctttatttgtaaccattataagctgcaataaacaagttaacaacaacaattgcattcattttatgtttcaggttcagggggaggtgtgggaggttttttaaagcaagtaaaacctctacaaatgtggtaaaatcgataaggatccgtcgaccgatgcccttgagagccttcaacccagtcagctccttccggtgggcgcggggcatgactatcgtcgccgcacttatgactgtcttctttatcatgcaactcgtaggacaggtgccggcagcgctcttccgcttcctcgctcactgactcgctgcgctcggtcgttcggctgcggcgagcggtatcagctcactcaaaggcggtaatacggttatccacagaatcaggggataacgcaggaaagaacatgtgagcaaaaggccagcaaaaggccaggaaccgtaaaaaggccgcgttgctggcgtttttccataggctccgcccccctgacgagcatcacaaaaatcgacgctcaagtcagaggtggcgaaacccgacaggactataaagataccaggcgtttccccctggaagctccctcgtgcgctctcctgttccgaccctgccgcttaccggatacctgtccgcctttctcccttcgggaagcgtggcgctttctcatagctcacgctgtaggtatctcagttcggtgtaggtcgttcgctccaagctgggctgtgtgcacgaaccccccgttcagcccgaccgctgcgccttatccggtaactatcgtcttgagtccaacccggtaagacacgacttatcgccactggcagcagccactggtaacaggattagcagagcgaggtatgtaggcggtgctacagagttcttgaagtggtggcctaactacggctacactagaagaacagtatttggtatctgcgctctgctgaagccagttaccttcggaaaaagagttggtagctcttgatccggcaaacaaaccaccgctggtagcggtggtttttttgtttgcaagcagcagattacgcgcagaaaaaaaggatctcaagaagatcctttgatcttttctacggggtctgacgctcagtggaacgaaaactcacgttaagggattttggtcatgagattatcaaaaaggatcttcacctagatccttttaaattaaaaatgaagttttaaatcaatctaaagtatatatgagtaaacttggtctgacagcggccgcaaatgctaaaccactgcagtggttaccagtgcttgatcagtgaggcaccgatctcagcgatctgcctatttcgttcgtccatagtggcctgactccccgtcgtgtagatcactacgattcgtgagggcttaccatcaggccccagcgcagcaatgatgccgcgagagccgcgttcaccggcccccgatttgtcagcaatgaaccagccagcagggagggccgagcgaagaagtggtcctgctactttgtccgcctccatccagtctatgagctgctgtcgtgatgctagagtaagaagttcgccagtgagtagtttccgaagagttgtggccattgctactggcatcgtggtatcacgctcgtcgttcggtatggcttcgttcaactctggttcccagcggtcaagccgggtcacatgatcacccatattatgaagaaatgcagtcagctccttagggcctccgatcgttgtcagaagtaagttggccgcggtgttgtcgctcatggtaatggcagcactacacaattctcttaccgtcatgccatccgtaagatgcttttccgtgaccggcgagtactcaaccaagtcgttttgtgagtagtgtatacggcgaccaagctgctcttgcccggcgtctatacgggacaacaccgcgccacatagcagtactttgaaagtgctcatcatcgggaatcgttcttcggggcggaaagactcaaggatcttgccgctattgagatccagttcgatatagcccactcttgcacccagttgatcttcagcatcttttactttcaccagcgtttcggggtgtgcaaaaacaggcaagcaaaatgccgcaaagaagggaatgagtgcgacacgaaaatgttggatgctcatactcgtcctttttcaatattattgaagcatttatcagggttactagtacgtctctcaaggataagtaagtaatattaaggtacgggaggtattggacaggccgcaataaaatatctttattttcattacatctgtgtgttggttttttgtgtgaatcgatagtactaacatacgctctccatcaaaacaaaacgaaacaaaacaaactagcaaaataggctgtccccagtgcaagtgcaggtgccagaacatttctct

SEQ ID NO: 32 - DNA, 5697 bp, Artificial Sequence
  reporter vector (E. coli)
ggcctaactggccggtacctagttattaatagtaatcaattacggggtcattagttcatagcccatatatggagttccgcgttacataacttacggtaaatggcccgcctggctgaccgcccaacgacccccgcccattgacgtcaataatgacgtatgttcccatagtaacgccaatagggactttccattgacgtcaatgggtggagtatttacggtaaactgcccacttggcagtacatcaagtgtatcatatgccaagtacgccccctattgacgtcaatgacggtaaatggcccgcctggcattatgcccagtacatgaccttatgggactttcctacttggcagtacatctacgtattagtcatcgctattaccatggtgatgcggttttggcagtacatcaatgggcgtggatagcggtttgactcacggggatttccaagtctccaccccattgacgtcaatgggagtttgttttggcaccaaaatcaacgggactttccaaaatgtcgtaacaactccgccccattgacgcaaatgggcggtaggcgtgtacggtgggaggtctatataagcagagctggtttagtgaaccgtcagatccgctagcgctaccggactcagatctcgagctcaagcttggcaatccggtactgttggtaaagccaccatggaagatgccaaaaacattaagaagggcccagcgccattctacccactcgaagacgggaccgccggcgagcagctgcacaaagccatgaagcgctacgccctggtgcccggcaccatcgcctttaccgacgcacatatcgaggtggacattacctacgccgagtacttcgagatgagcgttcggctggcagaagctatgaagcgctatgggctgaatacaaaccatcggatcgtggtgtgcagcgagaatagcttgcagttcttcatgcccgtgttgggtgccctgttcatcggtgtggctgtggccccagctaacgacatctacaacgagcgcgagctgctgaacagcatgggcatcagccagcccaccgtcgtattcgtgagcaagaaagggctgcaaaagatcctcaacgtgcaaaagaagctaccgatcatacaaaagatcatcatcatggatagcaagaccgactaccagggcttccaaagcatgtacaccttcgtgacttcccatttgccacccggcttcaacgagtacgacttcgtgcccgagagcttcgaccgggacaaaaccatcgccctgatcatgaacagtagtggcagtaccggattgcccaagggcgtagccctaccgcaccgcaccgcttgtgtccgattcagtcatgcccgcgaccccatcttcggcaaccagatcatccccgacaccgctatcctcagcgtggtgccatttcaccacggcttcggcatgttcaccacgctgggctacttgatctgcggctttcgggtcgtgctcatgtaccgcttcgaggaggagctattcttgcgcagcttgcaagactataagattcaatctgccctgctggtgcccacactatttagcttcttcgctaagagcactctcatcgacaagtacgacctaagcaacttgcacgagatcgccagcggcggggcgccgctcagcaaggaggtaggtgaggccgtggccaaacgcttccacctaccaggcatccgccagggctacggcctgacagaaacaaccagcgccattctgatcacccccgaaggggacgacaagcctggcgcagtaggcaaggtggtgcccttcttcgaggctaaggtggtggacttggactagggtctctgtcggataagagcacaaatatcatcgctcaaaccacttacggaggtaccgtgagacctaggagcgcgagctgctgaacagcatgggcatcagccagcccaccgtcgtattcgtgagcaagaaagggctgcaaaagatcctcaacgtgcaaaagaagctaccgatcatacaaaagatcatcatcatggatagcaagaccgactaccagggcttccaaagcatgtacaccttcgtgacttcccatttgccacccggcttcaacgagtacgacttcgtgcccgagagcttcgaccgggacaaaaccatcgccctgatcatgaacagtagtggcagtaccggattgcccaagggcgtagccctaccgcaccgcaccgcttgtgtccgattcagtcatgcccgcgaccccatcttcggcaaccagatcatccccgacaccgctatcctcagcgtggtgccatttcaccacggcttcggcatgttcaccacgctgggctacttgatctgcggctttcgggtcgtgctcatgtaccgcttcgaggaggagctattcttgcgcagcttgcaagactataagattcaatctgccctgctggtgcccacactatttagcttcttcgctaagagcactctcatcgacaagtacgacctaagcaacttgcacgagatcgccagcggcggggcgccgctcagcaaggaggtaggtgaggccgtggccaaacgcttccacctaccaggcatccgccagggctacggcctgacagaaacaaccagcgccattctgatcacccccgaaggggacgacaagcctggcgcagtaggcaaggtggtgcccttcttcgaggctaaggtggtggacttggacaccggtaagacactgggtgtgaaccagcgcggcgagctgtgcgtccgtggccccatgatcatgagcggctacgttaacaaccccgaggctacaaacgctctcatcgacaaggacggctggctgcacagcggcgacatcgcctactgggacgaggacgagcacttcttcatcgtggaccggctgaagagcctgatcaaatacaagggctaccaggtagccccagccgaactggagagcatcctgctgcaacaccccaacatcttcgacgccggggtcgccggcctgcccgacgacgatgccggcgagctgcccgccgcagtcgtcgtgctggaacacggtaaaaccatgaccgagaaggagatcgtggactatgtggccagccaggttacaaccgccaagaagctgcgcggtggtgttgtgttcgtggacgaggtgcctaaaggactgaccggcaagttggacgcccgcaagatccgcgagattctcattaaggccaagaagggcggcaagatcgccgtgaattcttaactgcagtctagagtcggggcggccggccgcttcgagcagacatgataagatacattgatgagtttggacaaaccacaactagaatgcagtgaaaaaaatgctttatttgtgaaatttgtgatgctattgctttatttgtaaccattataagctgcaataaacaagttaacaacaacaattgcattcattttatgtttcaggttcagggggaggtgtgggaggttttttaaagcaagtaaaacctctacaaatgtggtaaaatcgataaggatccgtcgaccgatgcccttgagagccttcaacccagtcagctccttccggtgggcgcggggcatgactatcgtcgccgcacttatgactgtcttctttatcatgcaactcgtaggacaggtgccggcagcgctcttccgcttcctcgctcactgactcgctgcgctcggtcgttcggctgcggcgagcggtatcagctcactcaaaggcggtaatacggttatccacagaatcaggggataacgcaggaaagaacatgtgagcaaaaggccagcaaaaggccaggaaccgtaaaaaggccgcgttgctggcgtttttccataggctccgcccccctgacgagcatcacaaaaatcgacgctcaagtcagaggtggcgaaacccgacaggactataaagataccaggcgtttccccctggaagctccctcgtgcgctctcctgttccgaccctgccgcttaccggatacctgtccgcctttctcccttcgggaagcgtggcgctttctcatagctcacgctgtaggtatctcagttcggtgtaggtcgttcgctccaagctgggctgtgtgcacgaaccccccgttcagcccgaccgctgcgccttatccggtaactatcgtcttgagtccaacccggtaagacacgacttatcgccactggcagcagccactggtaacaggattagcagagcgaggtatgtaggcggtgctacagagttcttgaagtggtggcctaactacggctacactagaagaacagtatttggtatctgcgctctgctgaagccagttaccttcggaaaaagagttggtagctcttgatccggcaaacaaaccaccgctggtagcggtggtttttttgtttgcaagcagcagattacgcgcagaaaaaaaggatctcaagaagatcctttgatcttttctacggggtctgacgctcagtggaacgaaaactcacgttaagggattttggtcatgagattatcaaaaaggatcttcacctagatccttttaaattaaaaatgaagttttaaatcaatctaaagtatatatgagtaaacttggtctgacagcggccgcaaatgctaaaccactgcagtggttaccagtgcttgatcagtgaggcaccgatctcagcgatctgcctatttcgttcgtccatagtggcctgactccccgtcgtgtagatcactacgattcgtgagggcttaccatcaggccccagcgcagcaatgatgccgcgagagccgcgttcaccggcccccgatttgtcagcaatgaaccagccagcagggagggccgagcgaagaagtggtcctgctactttgtccgcctccatccagtctatgagctgctgtcgtgatgctagagtaagaagttcgccagtgagtagtttccgaagagttgtggccattgctactggcatcgtggtatcacgctcgtcgttcggtatggcttcgttcaactctggttcccagcggtcaagccgggtcacatgatcacccatattatgaagaaatgcagtcagctccttagggcctccgatcgttgtcagaagtaagttggccgcggtgttgtcgctcatggtaatggcagcactacacaattctcttaccgtcatgccatccgtaagatgcttttccgtgaccggcgagtactcaaccaagtcgttttgtgagtagtgtatacggcgaccaagctgctcttgcccggcgtctatacgggacaacaccgcgccacatagcagtactttgaaagtgctcatcatcgggaatcgttcttcggggcggaaagactcaaggatcttgccgctattgagatccagttcgatatagcccactcttgcacccagttgatcttcagcatcttttactttcaccagcgtttcggggtgtgcaaaaacaggcaagcaaaatgccgcaaagaagggaatgagtgcgacacgaaaatgttggatgctcatactcgtcctttttcaatattattgaagcatttatcagggttactagtacgtctctcaaggataagtaagtaatattaaggtacgggaggtattggacaggccgcaataaaatatctttattttcattacatctgtgtgttggttttttgtgtgaatcgatagtactaacatacgctctccatcaaaacaaaacgaaacaaaacaaactagcaaaataggctgtccccagtgcaagtgcaggtgccagaacatttctct

SEQ ID NO: 33 - DNA, 3391 bp, Artificial Sequence
  crRNA vector (CCR5)
gtggcacttttcggggaaatgtgcgcggaacccctatttgtttatttttctaaatacattcaaatatgtatccgctcatgagacaataaccctgataaatgcttcaataatattgaaaaaggaagagtatgagtattcaacatttccgtgtcgcccttattcccttttttgcggcattttgccttcctgtttttgctcacccagaaacgctggtgaaagtaaaagatgctgaagatcagttgggtgcacgagtgggttacatcgaactggatctcaacagcggtaagatccttgagagttttcgccccgaagaacgttttccaatgatgagcacttttaaagttctgctatgtggcgcggtattatcccgtattgacgccgggcaagagcaactcggtcgccgcatacactattctcagaatgacttggttgagtactcaccagtcacagaaaagcatcttacggatggcatgacagtaagagaattatgcagtgctgccataaccatgagtgataacactgcggccaacttacttctgacaacgatcggaggaccgaaggagctaaccgcttttttgcacaacatgggggatcatgtaactcgccttgatcgttgggaaccggagctgaatgaagccataccaaacgacgagcgtgacaccacgatgcctgtagcaatggcaacaacgttgcgcaaactattaactggcgaactacttactctagcttcccggcaacaattaatagactggatggaggcggataaagttgcaggaccacttctgcgctcggcccttccggctggctggtttattgctgataaatctggagccggtgagcgtgggtctcgcggtatcattgcagcactggggccagatggtaagccctcccgtatcgtagttatctacacgacggggagtcaggcaactatggatgaacgaaatagacagatcgctgagataggtgcctcactgattaagcattggtaactgtcagaccaagtttactcatatatactttagattgatttaaaacttcatttttaatttaaaaggatctaggtgaagatcctttttgataatctcatgaccaaaatcccttaacgtgagttttcgttccactgagcgtcagaccccgtagaaaagatcaaaggatcttcttgagatcctttttttctgcgcgtaatctgctgcttgcaaacaaaaaaaccaccgctaccagcggtggtttgtttgccggatcaagagctaccaactctttttccgaaggtaactggcttcagcagagcgcagataccaaatactgtccttctagtgtagccgtagttaggccaccacttcaagaactctgtagcaccgcctacatacctcgctctgctaatcctgttaccagtggctgctgccagtggcgataagtcgtgtcttaccgggttggactcaagacgatagttaccggataaggcgcagcggtcgggctgaacggggggttcgtgcacacagcccagcttggagcgaacgacctacaccgaactgagatacctacagcgtgagctatgagaaagcgccacgcttcccgaagggagaaaggcggacaggtatccggtaagcggcagggtcggaacaggagagcgcacgagggagcttccagggggaaacgcctggtatctttatagtcctgtcgggtttcgccacctctgacttgagcgtcgatttttgtgatgctcgtcaggggggcggagcctatggaaaaacgccagcaacgcggcctttttacggttcctggccttttgctggccttttgctcacatgttctttcctgcgttatcccctgattctgtggataaccgtattaccgcctttgagtgagctgataccgctcgccgcagccgaacgaccgagcgcagcgagtcagtgagcgaggaagcggaagagcgcccaatacgcaaaccgcctctccccgcgcgttggccgattcattaatgcagctggcacgacaggtttcccgactggaaagcgggcagtgagcgcaacgcaattaatgtgagttagctcactcattaggcaccccaggctttacactttatgcttccggctcgtatgttgtgtggaattgtgagcggataacaatttcacacaggaaacagctatgaccatgattacgccaagcgcgcaattaaccctcactaaagggaacaaaagctgggtaccgggccccccctcgaggtcgacggtatcgataagcttgatatcgaattgacgtgaattcttcccatgattccttcatatttgcatatacgatacaaggctgttagagagataattggaattaatttgactgtaaacacaaagatattagtacaaaatacgtgacgtagaaagtaataatttcttgggtagtttgcagttttaaaattatgttttaaaatggactatcatatgcttaccgtaacttgaaagtatttcgatttcttggctttatatatcttgtggaaaggacgtggatgtgttgtttgtgtgatactataaagttggtagattgtgactggcttaaaaaatcattaattaataataggttatgtttagagtgttccccgcgccagcggggataaaccgtccaatctatgacatcaattattatacatcgggtgttccccgcgccagcggggataaaccgttttttgaattcctgcagcccgggggatccactagttctagagcggccgccaccgcggtggagctccaattcgccctatagtgagtcgtattacgcgcgctcactggccgtcgttttacaacgtcgtgactgggaaaaccctggcgttacccaacttaatcgccttgcagcacatccccctttcgccagctggcgtaatagcgaagaggcccgcaccgatcgcccttcccaacagttgcgcagcctgaatggcgaatgggacgcgccctgtagcggcgcattaagcgcggcgggtgtggtggttacgcgcagcgtgaccgctacacttgccagcgccctagcgcccgctcctttcgctttcttcccttcctttctcgccacgttcgccggctttccccgtcaagctctaaatcgggggctccctttagggttccgatttagtgctttacggcacctcgaccccaaaaaacttgattagggtgatggttcacgtagtgggccatcgccctgatagacggtttttcgccctttgacgttggagtccacgttctttaatagtggactcttgttccaaactggaacaacactcaaccctatctcggtctattcttttgatttataagggattttgccgatttcggcctattggttaaaaaatgagctgatttaacaaaaatttaacgcgaattttaacaaaatattaacgcttacaatttag

SEQ ID NO: 34 - DNA, 3391 bp, Artificial Sequence
  crRNA vector (E. coli)
gtggcacttttcggggaaatgtgcgcggaacccctatttgtttatttttctaaatacattcaaatatgtatccgctcatgagacaataaccctgataaatgcttcaataatattgaaaaaggaagagtatgagtattcaacatttccgtgtcgcccttattcccttttttgcggcattttgccttcctgtttttgctcacccagaaacgctggtgaaagtaaaagatgctgaagatcagttgggtgcacgagtgggttacatcgaactggatctcaacagcggtaagatccttgagagttttcgccccgaagaacgttttccaatgatgagcacttttaaagttctgctatgtggcgcggtattatcccgtattgacgccgggcaagagcaactcggtcgccgcatacactattctcagaatgacttggttgagtactcaccagtcacagaaaagcatcttacggatggcatgacagtaagagaattatgcagtgctgccataaccatgagtgataacactgcggccaacttacttctgacaacgatcggaggaccgaaggagctaaccgcttttttgcacaacatgggggatcatgtaactcgccttgatcgttgggaaccggagctgaatgaagccataccaaacgacgagcgtgacaccacgatgcctgtagcaatggcaacaacgttgcgcaaactattaactggcgaactacttactctagcttcccggcaacaattaatagactggatggaggcggataaagttgcaggaccacttctgcgctcggcccttccggctggctggtttattgctgataaatctggagccggtgagcgtgggtctcgcggtatcattgcagcactggggccagatggtaagccctcccgtatcgtagttatctacacgacggggagtcaggcaactatggatgaacgaaatagacagatcgctgagataggtgcctcactgattaagcattggtaactgtcagaccaagtttactcatatatactttagattgatttaaaacttcatttttaatttaaaaggatctaggtgaagatcctttttgataatctcatgaccaaaatcccttaacgtgagttttcgttccactgagcgtcagaccccgtagaaaagatcaaaggatcttcttgagatcctttttttctgcgcgtaatctgctgcttgcaaacaaaaaaaccaccgctaccagcggtggtttgtttgccggatcaagagctaccaactctttttccgaaggtaactggcttcagcagagcgcagataccaaatactgtccttctagtgtagccgtagttaggccaccacttcaagaactctgtagcaccgcctacatacctcgctctgctaatcctgttaccagtggctgctgccagtggcgataagtcgtgtcttaccgggttggactcaagacgatagttaccggataaggcgcagcggtcgggctgaacggggggttcgtgcacacagcccagcttggagcgaacgacctacaccgaactgagatacctacagcgtgagctatgagaaagcgccacgcttcccgaagggagaaaggcggacaggtatccggtaagcggcagggtcggaacaggagagcgcacgagggagcttccagggggaaacgcctggtatctttatagtcctgtcgggtttcgccacctctgacttgagcgtcgatttttgtgatgctcgtcaggggggcggagcctatggaaaaacgccagcaacgcggcctttttacggttcctggccttttgctggccttttgctcacatgttctttcctgcgttatcccctgattctgtggataaccgtattaccgcctttgagtgagctgataccgctcgccgcagccgaacgaccgagcgcagcgagtcagtgagcgaggaagcggaagagcgcccaatacgcaaaccgcctctccccgcgcgttggccgattcattaatgcagctggcacgacaggtttcccgactggaaagcgggcagtgagcgcaacgcaattaatgtgagttagctcactcattaggcaccccaggctttacactttatgcttccggctcgtatgttgtgtggaattgtgagcggataacaatttcacacaggaaacagctatgaccatgattacgccaagcgcgcaattaaccctcactaaagggaacaaaagctgggtaccgggccccccctcgaggtcgacggtatcgataagcttgatatcgaattgacgtgaattcttcccatgattccttcatatttgcatatacgatacaaggctgttagagagataattggaattaatttgactgtaaacacaaagatattagtacaaaatacgtgacgtagaaagtaataatttcttgggtagtttgcagttttaaaattatgttttaaaatggactatcatatgcttaccgtaacttgaaagtatttcgatttcttggctttatatatcttgtggaaaggacgtggatgtgttgtttgtgtgatactataaagttggtagattgtgactggcttaaaaaatcattaattaataataggttatgtttagagtgttccccgcgccagcggggataaaccgagcacaaatatcatcgctcaaaccacttacgggtgttccccgcgccagcggggataaaccgttttttgaattcctgcagcccgggggatccactagttctagagcggccgccaccgcggtggagctccaattcgccctatagtgagtcgtattacgcgcgctcactggccgtcgttttacaacgtcgtgactgggaaaaccctggcgttacccaacttaatcgccttgcagcacatccccctttcgccagctggcgtaatagcgaagaggcccgcaccgatcgcccttcccaacagttgcgcagcctgaatggcgaatgggacgcgccctgtagcggcgcattaagcgcggcgggtgtggtggttacgcgcagcgtgaccgctacacttgccagcgccctagcgcccgctcctttcgctttcttcccttcctttctcgccacgttcgccggctttccccgtcaagctctaaatcgggggctccctttagggttccgatttagtgctttacggcacctcgaccccaaaaaacttgattagggtgatggttcacgtagtgggccatcgccctgatagacggtttttcgccctttgacgttggagtccacgttctttaatagtggactcttgttccaaactggaacaacactcaaccctatctcggtctattcttttgatttataagggattttgccgatttcggcctattggttaaaaaatgagctgatttaacaaaaatttaacgcgaattttaacaaaatattaacgcttacaatttag

SEQ ID NO: 35 - DNA, 3391 bp, Artificial Sequence
  crRNA vector (EMX1)
gtggcacttttcggggaaatgtgcgcggaacccctatttgtttatttttctaaatacattcaaatatgtatccgctcatgagacaataaccctgataaatgcttcaataatattgaaaaaggaagagtatgagtattcaacatttccgtgtcgcccttattcccttttttgcggcattttgccttcctgtttttgctcacccagaaacgctggtgaaagtaaaagatgctgaagatcagttgggtgcacgagtgggttacatcgaactggatctcaacagcggtaagatccttgagagttttcgccccgaagaacgttttccaatgatgagcacttttaaagttctgctatgtggcgcggtattatcccgtattgacgccgggcaagagcaactcggtcgccgcatacactattctcagaatgacttggttgagtactcaccagtcacagaaaagcatcttacggatggcatgacagtaagagaattatgcagtgctgccataaccatgagtgataacactgcggccaacttacttctgacaacgatcggaggaccgaaggagctaaccgcttttttgcacaacatgggggatcatgtaactcgccttgatcgttgggaaccggagctgaatgaagccataccaaacgacgagcgtgacaccacgatgcctgtagcaatggcaacaacgttgcgcaaactattaactggcgaactacttactctagcttcccggcaacaattaatagactggatggaggcggataaagttgcaggaccacttctgcgctcggcccttccggctggctggtttattgctgataaatctggagccggtgagcgtgggtctcgcggtatcattgcagcactggggccagatggtaagccctcccgtatcgtagttatctacacgacggggagtcaggcaactatggatgaacgaaatagacagatcgctgagataggtgcctcactgattaagcattggtaactgtcagaccaagtttactcatatatactttagattgatttaaaacttcatttttaatttaaaaggatctaggtgaagatcctttttgataatctcatgaccaaaatcccttaacgtgagttttcgttccactgagcgtcagaccccgtagaaaagatcaaaggatcttcttgagatcctttttttctgcgcgtaatctgctgcttgcaaacaaaaaaaccaccgctaccagcggtggtttgtttgccggatcaagagctaccaactctttttccgaaggtaactggcttcagcagagcgcagataccaaatactgtccttctagtgtagccgtagttaggccaccacttcaagaactctgtagcaccgcctacatacctcgctctgctaatcctgttaccagtggctgctgccagtggcgataagtcgtgtcttaccgggttggactcaagacgatagttaccggataaggcgcagcggtcgggctgaacggggggttcgtgcacacagcccagcttggagcgaacgacctacaccgaactgagatacctacagcgtgagctatgagaaagcgccacgcttcccgaagggagaaaggcggacaggtatccggtaagcggcagggtcggaacaggagagcgcacgagggagcttccagggggaaacgcctggtatctttatagtcctgtcgggtttcgccacctctgacttgagcgtcgatttttgtgatgctcgtcaggggggcggagcctatggaaaaacgccagcaacgcggcctttttacggttcctggccttttgctggccttttgctcacatgttctttcctgcgttatcccctgattctgtggataaccgtattaccgcctttgagtgagctgataccgctcgccgcagccgaacgaccgagcgcagcgagtcagtgagcgaggaagcggaagagcgcccaatacgcaaaccgcctctccccgcgcgttggccgattcattaatgcagctggcacgacaggtttcccgactggaaagcgggcagtgagcgcaacgcaattaatgtgagttagctcactcattaggcaccccaggctttacactttatgcttccggctcgtatgttgtgtggaattgtgagcggataacaatttcacacaggaaacagctatgaccatgattacgccaagcgcgcaattaaccctcactaaagggaacaaaagctgggtaccgggccccccctcgaggtcgacggtatcgataagcttgatatcgaattgacgtgaattcttcccatgattccttcatatttgcatatacgatacaaggctgttagagagataattggaattaatttgactgtaaacacaaagatattagtacaaaatacgtgacgtagaaagtaataatttcttgggtagtttgcagttttaaaattatgttttaaaatggactatcatatgcttaccgtaacttgaaagtatttcgatttcttggctttatatatcttgtggaaaggacgtggatgtgttgtttgtgtgatactataaagttggtagattgtgactggcttaaaaaatcattaattaataataggttatgtttagagtgttccccgcgccagcggggataaaccgcaggccaatggggaggacatcgatgtcacctcgtgttccccgcgccagcggggataaaccgttttttgaattcctgcagcccgggggatccactagttctagagcggccgccaccgcggtggagctccaattcgccctatagtgagtcgtattacgcgcgctcactggccgtcgttttacaacgtcgtgactgggaaaaccctggcgttacccaacttaatcgccttgcagcacatccccctttcgccagctggcgtaatagcgaagaggcccgcaccgatcgcccttcccaacagttgcgcagcctgaatggcgaatgggacgcgccctgtagcggcgcattaagcgcggcgggtgtggtggttacgcgcagcgtgaccgctacacttgccagcgccctagcgcccgctcctttcgctttcttcccttcctttctcgccacgttcgccggctttccccgtcaagctctaaatcgggggctccctttagggttccgatttagtgctttacggcacctcgaccccaaaaaacttgattagggtgatggttcacgtagtgggccatcgccctgatagacggtttttcgccctttgacgttggagtccacgttctttaatagtggactcttgttccaaactggaacaacactcaaccctatctcggtctattcttttgatttataagggattttgccgatttcggcctattggttaaaaaatgagctgatttaacaaaaatttaacgcgaattttaacaaaatattaacgcttacaatttag

SEQ ID NO: 36 - DNA, 61 bp, Artificial Sequence
  primer1 (Cse1)
gcaaagaattcagatctccaccatgcctaagaagaagagaaaagtgaacctgctgattgac

SEQ ID NO: 37 - DNA, 49 bp, Artificial Sequence
  primer2 (Cse1)
tcatcgatgcatctcgagttatccattagaaggtcctccctgtggcttc

SEQ ID NO: 38 - DNA, 61 bp, Artificial Sequence
  primer1 (Cse2)
gcaaagaattcagatctccaccatgcccaagaagaagcggaaggtggccgatgagatcgac

SEQ ID NO: 39 - DNA, 49 bp, Artificial Sequence
  primer2 (Cse2)
tcatcgatgcatctcgagttaggcgttcttatttgtggtcagcacgaag

SEQ ID NO: 40 - DNA, 61 bp, Artificial Sequence
  primer1 (Cas5)
gcaaagaattcagatctccaccatgcccaagaagaagcggaaggtgtccaatttcatcaac

SEQ ID NO: 41 - DNA, 49 bp, Artificial Sequence
  primer2 (Cas5)
tcatcgatgcatctcgagttatgcctctccattgttccgcacccagctc

SEQ ID NO: 42 - DNA, 61 bp, Artificial Sequence
  primer1 (Cas6)
gcaaagaattcagatctccaccatgcccaagaagaagcggaaagtgtacctgagcaaagtg

SEQ ID NO: 43 - DNA, 47 bp, Artificial Sequence
  primer2 (Cas6)
tcatcgatgcatctcgagttacagaggtgccagtgacagcagcccac

SEQ ID NO: 44 - DNA, 61 bp, Artificial Sequence
  primer1 (Cas7)
gcaaagaattcagatctccaccatgcccaagaagaagcggaaggtgcgctcctacctgatc

SEQ ID NO: 45 - DNA, 49 bp, Artificial Sequence
  primer2 (Cas7)
tcatcgatgcatctcgagttactggctcacgtccattcctcccttgatc

SEQ ID NO: 46 - DNA, 6265 bp, Homo sapiens
tcaccaaccgccaagagagcttgatatgactgtatatagtatagtcataaagaacctgaacttgaccatatacttatgtcatgtggaaaatttctcatagcttcagatagattatatctggagtgaagaatcctgccacctatgtatctggcatagtgtgagtcctcataaatgcttactggtttgaagggcaacaaaatagtgaacagagtgaaaatccccactaagatcctgggtccagaaaaagatgggaaacctgtttagctcacccgtgagcccatagttaaaactctttagacaacaggttgtttccgtttacagagaacaataatattgggtggtgagcatctgtgtgggggttggggtgggataggggatacggggagagtggagaaaaaggggacacagggttaatgtgaagtccaggatccccctctacatttaaagttggtttaagttggctttaattaatagcaactcttaagataatcagaattttcttaaccttttagccttactgttgaaaagccctgtgatcttgtacaaatcatttgcttcttggatagtaatttcttttactaaaatgtgggcttttgactagatgaatgtaaatgttcttctagctctgatatcctttattctttatattttctaacagattctgtgtagtgggatgagcagagaacaaaaacaaaataatccagtgagaaaagcccgtaaataaaccttcagaccagagatctattctctagcttattttaagctcaacttaaaaagaagaactgttctctgattcttttcgccttcaatacacttaatgatttaactccaccctccttcaaaagaaacagcatttcctacttttatactgtctatatgattgatttgcacagctcatctggccagaagagctgagacatccgttcccctacaagaaactctccccggtaagtaacctctcagctgcttggcctgttagttagcttctgagatgagtaaaagactttacaggaaacccatagaagacatttggcaaacaccaagtgctcatacaattatcttaaaatataatctttaagataaggaaagggtcacagtttggaatgagtttcagacggttataacatcaaagatacaaaacatgattgtgagtgaaagactttaaagggagcaatagtattttaataactaacaatccttacctctcaaaagaaagatttgcagagagatgagtcttagctgaaatcttgaaatcttatcttctgctaaggagaactaaaccctctccagtgagatgccttctgaatatgtgcccacaagaagttgtgtctaagtctggttctcttttttctttttcctccagacaagagggaagcctaaaaatggtcaaaattaatattaaattacaaacgccaaataaaattttcctctaatatatcagtttcatggcacagttagtatataattctttatggttcaaaattaaaaatgagcttttctaggggcttctctcagctgcctagtctaaggtgcagggagtttgagactcacagggtttaataagagaaaattctcagctagagcagctgaacttaaatagactaggcaagacagctggttataagactaaactacccagaatgcatgacattcatctgtggtggcagacgaaacattttttattatattatttcttgggtatgtatgacaactcttaattgtggcaactcagaaactacaaacacaaacttcacagaaaatgtgaggattttacaattggctgttgtcatctatgaccttccctgggacttgggcacccggccatttcactctgactacatcatgtcaccaaacatctgatggtcttgccttttaattctcttttcgaggactgagagggagggtagcatggtagttaagagtgcaggcttcccgcattcaaaatcggttgcttactagctgtgtggctttgagcaagttactcaccctctctgtgcttcaaggtccttgtctgcaaaatgtgaaaaatatttcctgcctcataaggttgccctaaggattaaatgaatgaatgggtatgatgcttagaacagtgattggcatccagtatgtgccctcgaggcctcttaattattactggcttgctcatagtgcatgttctttgtgggctaactctagcgtcaataaaaatgttaagactgagttgcagccgggcatggtggctcatgcctgtaatcccagcattctaggaggctgaggcaggaggatcgcttgagcccaggagttcgagaccagcctgggcaacatagtgtgatcttgtatctataaaaataaacaaaattagcttggtgtggtggcgcctgtagtccccagccacttggaggggtgaggtgagaggattgcttgagcccgggatggtccaggctgcagtgagccatgatcgtgccactgcactccagcctgggcgacagagtgagaccctgtctcacaacaacaacaacaacaacaaaaaggctgagctgcaccatgcttgacccagtttcttaaaattgttgtcaaagcttcattcactccatggtgctatagagcacaagattttatttggtgagatggtgctttcatgaattcccccaacagagccaagctctccatctagtggacagggaagctagcagcaaaccttcccttcactacaaaacttcattgcttggccaaaaagagagttaattcaatgtagacatctatgtaggcaattaaaaacctattgatgtataaaacagtttgcattcatggagggcaactaaatacattctaggactttataaaagatcactttttatttatgcacagggtggaacaagatggattatcaagtgtcaagtccaatctatgacatcaattattatacatcggagccctgccaaaaaatcaatgtgaagcaaatcgcagcccgcctcctgcctccgctctactcactggtgttcatctttggttttgtgggcaacatgctggtcatcctcatcctgataaactgcaaaaggctgaagagcatgactgacatctacctgctcaacctggccatctctgacctgtttttccttcttactgtccccttctgggctcactatgctgccgcccagtgggactttggaaatacaatgtgtcaactcttgacagggctctattttataggcttcttctctggaatcttcttcatcatcctcctgacaatcgataggtacctggctgtcgtccatgctgtgtttgctttaaaagccaggacggtcacctttggggtggtgacaagtgtgatcacttgggtggtggctgtgtttgcgtctctcccaggaatcatctttaccagatctcaaaaagaaggtcttcattacacctgcagctctcattttccatacagtcagtatcaattctggaagaatttccagacattaaagatagtcatcttggggctggtcctgccgctgcttgtcatggtcatctgctactcgggaatcctaaaaactctgcttcggtgtcgaaatgagaagaagaggcacagggctgtgaggcttatcttcaccatcatgattgtttattttctcttctgggctccctacaacattgtccttctcctgaacaccttccaggaattctttggcctgaataattgcagtagctctaacaggttggaccaagctatgcaggtgacagagactcttgggatgacgcactgctgcatcaaccccatcatctatgcctttgtcggggagaagttcagaaactacctcttagtcttcttccaaaagcacattgccaaacgcttctgcaaatgctgttctattttccagcaagaggctcccgagcgagcaagctcagtttacacccgatccactggggagcaggaaatatctgtgggcttgtgacacggactcaagtgggctggtgacccagtcagagttgtgcacatggcttagttttcatacacagcctgggctgggggtggggtgggagaggtcttttttaaaaggaagttactgttatagagggtctaagattcatccatttatttggcatctgtttaaagtagattagatcttttaagcccatcaattatagaaagccaaatcaaaatatgttgatgaaaaatagcaacctttttatctccccttcacatgcatcaagttattgacaaactctcccttcactccgaaagttccttatgtatatttaaaagaaagcctcagagaattgctgattcttgagtttagtgatctgaacagaaataccaaaattatttcagaaatgtacaactttttacctagtacaaggcaacatataggttgtaaatgtgtttaaaacaggtctttgtcttgctatggggagaaaagacatgaatatgattagtaaagaaatgacacttttcatgtgtgatttcccctccaaggtatggttaataagtttcactgacttagaaccaggcgagagacttgtggcctgggagagctggggaagcttcttaaatgagaaggaatttgagttggatcatctattgctggcaaagacagaagcctcactgcaagcactgcatgggcaagcttggctgtagaaggagacagagctggttgggaagacatggggaggaaggacaaggctagatcatgaagaaccttgacggcattgctccgtctaagtcatgagctgagcagggagatcctggttggtgttgcagaaggtttactctgtggccaaaggagggtcaggaaggatgagcatttagggcaaggagaccaccaacagccctcaggtcagggtgaggatggcctctgctaagctcaaggcgtgaggatgggaaggagggaggtattcgtaaggatgggaaggagggaggtattcgtgcagcatatgaggatgcagagtcagcagaactggggtggatttgggttggaagtgagggtcagagaggagtcagagagaatccctagtcttcaagcagattggagaaacccttgaaaagacatcaagcacagaaggaggaggaggaggtttaggtcaagaagaagatggattggtgtaaaaggatgggtctggtttgcagagcttgaacacagtctcacccagactccaggctgtctttcactgaatgcttctgacttcatagatttccttcccatcccagctgaaatactgaggggtctccaggaggagactagatttatgaatacacgaggtatgaggtctaggaacatacttcagctcacacatgagatctaggtgaggattgattacctagtagtcatttcatgggttgttgggaggattctatgaggcaaccacaggcagcatttagcacatactacacattcaataagcatcaaactcttagttactcattcagggatagcactgagcaaagcattgagcaaaggggtcccatagaggtgagggaagcctgaaaaactaagatgctgcctgcccagtgcacacaagtgtaggtatcattttctgcatttaaccgtcaataggcaaaggggggaagggacatattcatttggaaataagctgccttgagccttaaaacccacaaaagtacaatttaccagcctccgtatttcagactgaatgggggtggggggggcgccttaggtacttattccagatgccttctccagacaaaccagaagcaacagaaaaaatcgtctctccctccctttgaaatgaatataccccttagtgtttgggtatattcatttcaaagggagagagagaggtttttttctgttctgtctcatatgattgtgcacatacttgagactgttttgaatttgggggatggctaaaaccatcatagtacaggtaaggtgagggaatagtaagtggtgagaactactcagggaatgaaggtgtcagaataataagaggtgctactgactttctcagcctctgaatatgaacggtgagcattgtggctgtcagcaggaagcaacgaagggaaatgtctttccttttgctcttaagttgtggagagtgcaacagtagcataggaccctaccctctgggccaagtcaaagacattctgacatcttagtatttgcatattcttatgtatgtgaaagttacaaattgcttgaaagaaaatatgcatctaataaaaaacaccttctaaaataattcattatattcttgctctttcagtcaagtgtacatttagagaatagcacataaaactgccagagcattttataagcagctgttttcttccttagtgtgt

SEQ ID NO: 47 - DNA, 29 bp, Artificial Sequence
  primer1 (CCR5)
ccacttggaggggtgaggtgagaggattg

SEQ ID NO: 48 - DNA, 25 bp, Artificial Sequence
  primer2 (CCR5)
taaagatgattcctgggagagacgc

SEQ ID NO: 49 - DNA, 25545 bp, Homo sapiens
gcagtctttctgccacagcctcccaaagtgctgagattataggtgtgagccattgtacctggcttggagtaatgtttttgagcaaagcaaatgtacaggacatgcacagagaggcacagggagcacagagtccctggatgaatgctctggctggtggcagtattgtcacagggcaggctacccaaaggtgagcagaacacatgaggctagacaggtacaacttgctcatgaagagcctcgaatgccaagcttaggagtttgaactttattggaacactgacactaatagttaatgtttactgagtgcttactatgtgctaagagctatgcatgaatcacctcattctaattctcttaactctccacagcaggtcttattatttccagattgctgatgaaaaactgagtcacagagaggtaaaaaaaaaaaaacaaaaacaccctgggtccagagttgtgtgaaaaaattttaacaggttagagttgtgttgtagaaatctggtagccagccacgtgtaagacgaattgtagaaaggagagatcacaaatggctatcataagagaatcactgggaaaaggtaataagaacccaaattagaggcaaggagaacagaaagaaatgaaagaatgcaaagactgactggatgtgcacagcagtgaccgagagaaaggaggtatcacaggtgcctcttagctgctaagcctgggtgtcctgcagaaaggggcagctattatcagaagagagaagccagagagaggcacagatttggtggggatgatgttgagctccgtttgggggtatggtgagtgtctagggggcctgtaggaacccctccagaaaaattctcacaagcatttgaaaatcagtgacttgatctggagaaaaatatagggctggcattacaaacctgccggggtctgcattacagtattggttgaaagtgtggaaattgataatgatagatggttggtagatacatagatagatagatagatagatagatagatagatagatagatagatagatagatagaataaatagcatgatacatggaatgagggaagggctaaggataaagatgccttcatggatgcccacagttaggagaagaaagtagagcccatgaaggaacaactcccagagtttgcagatccaggcaagtatcttgttcagaaaataaagggaagggagtttccaaaagaaaagggggttgaaggtactcagatgctgaggagcctataaacaattgtgactaaaaaagactcaaatttggaaataaggtgtcctaatgaacatttcagaggatggagagagattcttaaagtcagcctttggaagaataactatatagaacacttccagaggccaaactagtgacaatggatcaaaagaattaaaatattgcatatctggaaattacacagctagaaatatgtagaaaagaaacacaaacatgcggtaagatacagctatggagctgtttgtcgaaattttgttaaaacagtgaaaatctgtaaactgtattaatgtccaacaataaaaaatatttaatgagaggcaaagatgctttgattggttataaagataaagaagttacaatactatgtacagtatgatcctttttttaaagggaggcacatatagaaagaactggaaggatatactgtaagaatttcacgatgtttgtttctgggtagtaggatttgacaattataagatctctgttttcccttcactccccccttttggattatctgtattttttataactctgtccaatagacatataatgtgagacacataattttaaatgttctagtggccacatttaaaaagtagaaagaaatagataaaataatcttcttaagatatttcattttactcaatatatccattactatgtgtaatcgatataaaaatattaatattttaaatgttttagcactaagcctgtttaacactaaatgcagtggatattcacatttacagaacatctctgtttgggccatccacttctcaagcaccacattaccgcatttggctcctagcacggctctatgaaataatagcagttaatatttatcaaaagcctactatgttccaggcactgctccaagttcatcaggtggagattataactcattaggtctcaataactccatgaggttgaacttattgtgctctccacaagcacgtgttgcttgcccttgtcctcataccataatgaaatgtttggagcttttgcaaaagccattttcctaatatgatgggcatccaagtctggttgcaaaggcttggatagagggcaagtgagagaattggagagagactaaaaatcattcaagaaattttgtggtgaaaaagacaagtcaaaagactgagagaaacatgaggacagaaaactctttgtaaggcaaggagacataaagatgaagtcaggctgaataggaaagaaggaggtgaaaggtgaaagagagatggctgggggtgtggctggtccaaattctcacaagatctctgttggagaaacattgcctggcttgtgctggtggcgagatgtacatagcagcttcccagctagagggagcagggagtcatggccttgtgagggagacagatggagacacacacaacccccatcgcaggtgaatgctatgaaagaatggggtggagggcttcccagggagatgaactgagttttaagaacgaagttagccagcaaagaagcaaaaggaagaggatatagacttgaggattacatcactggatgactgagccactgattggatgtggaggatgagagagtgatgctttgaggtgattcccaagttctccgcatggacaaaggcagagacaataacttgtactgagtgctctttggagtctgacattgatccagtgcaccacatatgttatctcatttactcctcacagaggtcccgtataacgcttgcaatttcacagatacgcaagctgaggcaaaataattggcccagggctcaccactaataaataggagagtctggatttggggccaggttattccagaaatagagagagggagggaaaacgttaatgtggggccagagccagaacaggtaggctaggctgtatcagcctgggaggcatcgggctattctccaaaaagtgaggctccgggttgcaggagatgggacctccaggaaactggtgggaggctggacaggggcaaagtgaaaggtaagcagcctgaagatgggtgggatgtagtggactccagcgtgaagagcctccagtctctggcagagctcagcagcttgggtgggaggaaacgaagggcagggagcagaaggtggtggggggaacgggttttggttaagatgggcagctgtccagtggtgaagaggggaagtatttgtgtatacgatcagttgtgggggatggtggtagagggagcagtatgagagtctgggaggaacagggcaggggagatggcacaggagaagattggggtgggggtgggggcactgatactgaatccagtacacagaggcaggcttagagaccccctgagggtgacaaattcttctcttaacttgctgcagaggaaacgacaagagaataggtcctaagaggagtgaaaatagaggaaactggccaagggataaagataagcagagctatggaagaaaaggaagaaaattagggaattactggagaggaagctgacagaaaggggcgctgggagaggaaaaggtgagggaggacgaaaacggaactcctatcacccagcgcattccagcaccccctccccctcccccgggaagtctgcgactgcatcctcacagggatggaatgggagtggaagctaggccaggctgggaccccggggctgtcccagcccaaccaagacggtgaccagactcaagttactgatcctccgctgtttcttcatctgtaaagtggagttaatgacagacagctggatgtcaacgttttttgttgtttgttttagagatgggatctccctgtatcgcccaggctggagtgcagcggtatgatcacggctcactgcagcctcgacctcctgggctcgagagatcttcctgtctcagcctcccgagtagaaatgtcagcatttgaatgcctcacaagggaaggtggtgtaataaaaggtctattgatttagatatgaacaagtatacccagagccacacgaatgaaaggaggtggccagtgtagatgcaagtctaggacggtcggtagattccaagcttctctacctgcccagttaaacaagttcgtggcccctggccagcctctcggtgggggtctgcgacagaacgggtgggattcattaccaggctaggagcgcaaggccctcgggccgggttcagcttgctgggctcctgtcttgtctcagcccccagcacttgctctgtcaccgcagagcacaggcccaggcaacgtttacccaactgaacccgcatccctgtgggaaccttgttccaacaaaatcccgtcgttgtctccttccatatggaacgaaaatctccttctgtacctctgcccagctccgcacccccgcccccttagagatacggcctggtcgggtcctggtccccccctcggcggcgcttccacttttcccagactgagggtggggaaaaggaggagggggaagaaatcagaggaggaaaagtcgggaggtaggggagccgggagacaggagagggggaaaataaagagcctgagacacaaacgagaggaaaagaccatcacagaaagctggaaatctccggagaggccagcgagaacccgcgctccccacggattccatcattccttccgaaggcgcctctgcggtgtctcagccgtgccaggccccggggttcccaggacgcggaggagtgctgggtgcggccgcctcgcctccccacccctggccgcccctccccacctcgcccaagggggccggaacggcgtcggcgcgcgggggcttttcggagcagtcgagtggaaaatagactttaacccgctttgtggcggccggggcgccctgagcgctctccaaaccacggctcccggcgctcaggcgggccgctgccaagacccggcctggagtccccgcagagttgcgcggcgcacggaccccgtggccttggggcgtcaggaggcccaacccagatctgcgcgcccaggcagcgctcaggccgctagaatggaccccggcagcggcgaggaagcggaactctctgcggctccctctccgcagtgcgccggcaaggtccaggtcccagcctccccaccgccgcccgcgccctcctaggcctcggagcggcgcctttctgcggcctcgaaggtggggtgggaaagtttggggagtcccggctctcacagcctgtcgtgagaactgcccccggggaattcgtccgccgtacggaaaaactggccggagcagagtcgtccgcggttccgcggtcgcgggtggaaggtgaaggtcgagggaggtcaggctgcttctgcgtgtcctgacggctggcgtgttctcttgagatgggctcgggctacttggccagcttcaatttaagccacagtgtctccgaggccctgacctggtccggcccgccgacacttgagcccccagagcctcagagaaggcgagggggtggatctcccagtgccgaggcccgccgtcctggtccaagccggtcgcggcaccgtgtctgggcactggagctgcttccagccccgcgaacagctggagggtggcagtgggaccgctccggcggcttctcccgcgcagtgccccgcctggccccttgtgaagggagtgagcgtcccctttccagagctgtcccccgtgacatccagaaaacgcgaaacctcaggaacaaggtcgcagcttcagaccgcggcccaggaggccgatggtgggtgagtgggagagtcccggagagcaggggggcagagagctggttttcgggaaaaccaatgtgttggaccccaaacatccaccctccgctcggatccaagttctctgagaactgaaacgacatcccgggacgaatgggagagttaggctgagctacacaccggggaggggagggttggagtttagccccaagcccttcggacgccttcttcggctcccgcgtgggttgagacggcggcacggccaccagactcagctaaagggcggagtcgcgaggagaagccagtggcgaggggaggaggaggcctggatctccccgcgaaggctccagtccggcttttgcctccgactgcgggctccctccccacccgccgtccctcgccccgccccgccccgccccccaccttggggcaggtgagcggcggccaatgggcgagcgcggggcaggtgcccgctaactcgcgcctcgcagcgctgggcggccggggctgggcagggcagtgcggggacaccgggggctggggtcggtcccagcgggactccgaaaggagggagacgagctcaaccctcgggccttactggcagctcgcagcctagcacggagcccgcgcctgtgcgggcgcctggagctgcccgctccgccgcagcagccgccgcgcctggccgtacgctgtggccggaccccgcggtcgctcgctcacacacccctcgccgctccgcgcctggctcgcccgcgggggccgagcgcgagcgggcgggcgggggaggtgaggggtgcgggcgggtgtgcatgtgcctggctgggtgcacaccccgcaaggcggcggcgccaggacgcggagcgctccccagagcccggctgcctcgcacagctcccgcggctgcgaccatgttccagcccgcggccaagcgcggctttaccatagagtccttggtggccaaggacggcggcaccggcgggggcactggcggcgggggcgcgggctcccatctcctggcggcggccgcctccgaggaaccgctccggcccacggcgctcaactaccctcaccccagcgcggccgaggcggccttcgtgagtggcttccctgccgcggccgccgcgggcgcgggccgctcgctctacggtgggcccgagctcgtgttccccgaggccatgaaccaccccgcgctgaccgtgcatccggcgcaccagctgggcgcctccccgctgcagcccccgcactccttcttcggcgcccagcaccgggaccctctccatttctacccctgggtcctgcggaaccgcttcttcggccaccgcttccagggtgagtgtccacgctgtgcccgccgaggcggccggccggcgcccgtgctgcggcgatgcgggggaggctcgggggcgcgcggggctgtttagaagttactgccgggaaggctgcaggtccgcggaggtagattcccaggcagggaagagctgtgcggcatccacccgcgccttcgccgcgtaggtctccctcccaggaaagcaggtggagacctccaggcttttctagaaaatataccagttcggacgcaagcccaggcgcgtcctcggagcctgtgctggccctcgccacagcctgcccaattctctctcccagctgagccagtctcagaccagagtacaactcctcccgctctccctccgcccggcttaacctcgcaccacgcttctctcgcaagtccaccaccacctccgagacctcagccttcgctggcgcgtccgggcgggggaaagtccattcgcgtgccccagctctgggggaagcaagggcagcagggagggcgaatcggagagttaatgttcagtgtggagggcctggctgtcttgggatgtttctcggcaaccttggcccgacttctccaagtcacacgtgcctctcctacccaaggtggggaaggtttgcagtaagcaaactggcttccgccgttgctcgccgccttcgggagggagcccacccggctgctggaataccgaggacagttttcccgggcagggggcgggggcagagggcttttaaggtcgtagccagtccgaaccccggagtttgcatccagcaatcggcttgctaataaagatcctccactggccctacacacacacacacacacacacacacacacacacacacgtttcaattatttgtctttcccggagaaaagagagttgcatttgttggagttcgttttcttccttgaaatttgttggagtttgtttttttcttttctttttttttaaattttattttaaagagtggccttgatttgtacaggcatcactttagtttccagttttattttgttagtgtagaccagaccacagccttgtgagaagggtctatggctcagagctaggtaacccggcttttagagaaacaaatgaaagggacatggctggagcttcggctccaggagctaatgtgacggtctgtagtctaggtctacagtcaattagatgtttggcacagttgtttagataataaaatgaaaattatctcttgacactttgactttcacagaaaaccgctttcccaggtcccgatttgtcaggcaattttttcagtcccacctggccaatagatgctgacctggcagataccacaaaaccagagaatgtaattactagaataagaattgttgtgggtagccttgcctcctctttgaagatttcaaagacttgcccaaatccaaatccgaaaaaacaaaaatgctacaatgtcatctgccttgggcaagagtttctgccacttaaaaataaatgtttactgataacatgaggatatctttaaaattgagcaatctaccctggtcctccgtgggctcgatccgaagcctgggtctcgaaacctggcgcccaggggccgagttgtagttggggcggtgtgtgagcccgcgggccgccgcggccgaggggctggcgggttggaggcttgtggagggataggggctcggaggagagggcggggtcgttcctaagtcctgtggcctccagccgttcagcttgtccggagtcggcatcctgggccgcaccctcggcttcgaatccagcccctgacgccctccgcaccgcggttcctgcctccgggcgccgagggccgggggcgcctggagagaaatccagctccggctctgagcgtctccagtcaggcgaggcggataaatccttcgcaaaaccctcttggaaattgccgccgcttcctgagccatcagtcccagcgggtacgttatcgagtagcacaaacagttggatttttccctcaagaaccgagtctggacgcggagatggagccaagtgtggctgcattttcggacccggaaatccgttgggcactgaaggacttttcgaaccctgtagcgctgttgcttcgcggtccatcgtcgccgctgcagacggatgcgctccccggcggctctacgccctccagtcccggccaggcctctgggctgggagccgagccgtctcgggccctccggcgccgcgttttctagagaaccgggtctcagcgatgctcatttcagccccgtcttaatgcaacaaacgaaaccccacacgaacgaaaaggaacatgtctgcgctctctgcgcagcgcttgggcggcgcggtcccggcgcgcggggaagcggcgtctccgctaaccgaggcgctggaaggggaaaagcgaatgcggaatcgtccaggactccgaaggtcggggccgctcgcgagcaccgaaggggaggagccgacgaagaccaggagtgggccgcatttcggtactgtttccccgagatcaggaactttccgggtctaggagcaacgcctggagggggctgtagagacccagccccccgggacccgcaactacaatgggccggagcttctaaggtcgcctttgttctggcaggaggacggggaatgaggttatctccgccgcctgtcctgcctctccctctcctagccctagggccctccgcccagccgtccggccctgagcccctggccggcggcggcctctccagcgaagactgcggctcgaagactgcagctcggaccccgggtgcttcggatccctagctcccacctccagctccctcattcctgggaatctcttgtgctagttcccagccattgccttgaaggggccctaaaagagtggctgtagaaaaatcggaggggtagggaagcagggaggagaggggtattcatttccctagctccagggacggctataccagtccctttccactttgctaactgtcctagtccgaaactgacagcccgttctcacagcccagaattactgcgtccaaacaggccgcaccctagacccaagtttgttctgcccttgtggtccaggcaagggaaactgaacccctggtaggggtggttcaggcctccttcccacaggtcggggggcggggcggtacaggtacctgtgcacctaaggcatcacccttgtctttgcagaaacatgtagcaattgatctgtttctcaggatgtttggtgttgtactaaacatcctctttctaacagggaaacgtccttattcttttggaatcaaataacctgtcatcacttagcatcttgactcatcctgcagtctcctgcttctctgtgatagggttagaaggacccctgtatttttgcacatgcatgtgaatataccctttaggacacatgctgtctaccacaactggacatgacaatgacctggggccattttctcagtaaggtagacccaaagcaacctagcatccccctaaaataaccagacttgaggcaaaggggcatgtatgttggtacagaagcttgttgccttcatcctctcatctgggtttataaagacaaacacagagcactccaccacacaggtgactgacatataccacataattacaaaataatcactaagtcagagacactggggcagactgcagacctgcttcctcagccccacactgcccttcacacctctgcctcctattcatacacacttacggggctttccacactgcagcctcacttctgaccaacctgggccagcccagcatctgaggccaaaccctgccaatgctgggatgagctaggctttctctctccctctctggttcatttgtccagaggaaaccactgttgggacttcacccaggttcataacaatgttgttttttgaagcaagttattaacattaacaagaagcatttgctttccacccacctttccctggcctacctcactggccccaccccagagactttaatcttccttattccccacctggagcaggctccatatttttctgccctttactcatctctgccagaccacctcccctgaccatctgtctattccactatcccaagtcaaacttctcttcagtcggacctgagggccctagatctgcgccacttgaataatcaaatggggtgtccctcacccatctccctgtgatgtggtcccaccatttttgtggctgcacagatccaaccagttgaaattgataaggtgactggagattattgactgaccccttccaggcactagccccgcaatcctagcaactctgttccacagaaaactccagcaaaaacttggcttctttaggtaaccaaagcccagagacttggaggaagtaaggtcagggagtttccaccaacagagggacaagaacagttacctggagagttttagctacagcatctcaattatctgcttttgattcacttacatagatgtttccagagatgggagatgttaactgaattatccaggtgattgtcttagagcaaagcaacaggtcaaatcaagtccaaccagtagccatctctgaagaaattaattggatcagtcaatcccaacagctaattctgtcaaaataatccatctagggttccgtgtttttggtgcatcaggaggctgttatgtgcccttacatgagaatccatgggtgattttgtcagggcctgttatgagtctgttagcatgtgcaaccaagccagagattgtgtgagggcctagtggggtgttcattgagacaggcgctgtgggtagaggcttgttttggcattgatagtttctgaccccatctcccctaccccagcttcatccagtccagtgttatcccttcctcctgcatgtgggagctgagtccctatgctggccaacatttgctaagggacagtcacactctaaaaatcctatacagtagataggaaaaaagacagtagggaggctggaacatatatttacacacgcccatgcagaaaccaatatatctatatctatatatattagagagaaagatgacatctagatatttatacacatgtttctttagcaagggactattcagggatgaagcagggatgaagcttttcccaccagacagtacttggagtctccagtgtgtgtgttgggatagggggttgggggcttaccctagaggctgggtctctggaccgccaaggcctgggggagagagaggtggagaaaggggaagaaggagcctgactttccacttccaggtgctgcctggaccactgacctagccactggcctatttataccccctgcaagacagagctagagcgtgctggcaggagtttttaatgagttagtagcctgagcattcagccgcaagactagtgcaagcaggtgtgaagggattgctccttgtgtaccttctagttcttgaatctgtgtttggcaaaggtgtgcctagcaccccgctgctccccttatcacgttcctgacccccagccctgcctctaccctgggtcctcttggagggagatgctttgcgaccagttaactgaaagcaaatcgttggggctggcggccagggcagcgcccctgggaaagggcggagaaagagcgccatggacttttcttccccaccccttggcctcttccgctgccccaggcattgtgaatgtgggtccacgcctcgtccggcctgccccatctcttggcttaacagagggatctggagagctgttattccccgcgttcccccgcggagtggctctcgagtgcggggaggtgttgcggaggggagtggacttagggaaggggcggcaaaagggcaaagggagaaatggcgtgtgtgtgcgtgtcaaggaatggagagggcagggcgcttgggagcagggcgcgaggccaggctctgttgggccccggctcacggcgccccttctctctgtctgtacctgcgtgtgttgccgtcggcggcggggccgcagccagcgacgtgccccaggacgggctgcttctgcacggccccttcgcacgcaagcccaagcggatccgcacggccttctcgccctcgcagctgctgcggctggagcgcgccttcgagaagaaccactacgtggtgggcgccgagcggaagcagctggccggcagtctcagcctctccgagacgcaggtaatcacccccggtcgcggcctgccctgcgcccggagcccgggtggaggtgagggtgcgcgggtgcaggagaggccctgagcccgccccagcccagccctgctgggttccaaaaggcccccattccccgcggcgctgcggtcaagcccgtctttagagcctcttcctcgagactgcgtgcagcctgctgagcccgcaggacttttgtcaagcgctaaagacctagcaggaggcagagtaaatgcaaactgtatcccgagcccggctcccaaagctcctcacggggggaccaggttccctggaggaagcgggtcgcctcgggagcgggcagcgcaggcagcaccgaggccactggagctggctccagccctggcattcctgcagcccttttcccgccactgtgtcggggcgctcatagtcctgcggggagccggtccgcactggctttgctgctgttcctgggcaaaactggcggggccttggctgcccaccagccaggagcgtctggggagaaagcccaggtgtcctcagactaccaacagaggggcttaaccagggaggggccagcccctgcttggggcccgagggttgctctgatccggcccaggccggctgatagggctgtggaagccacggtgtgcgcgcgcagagcatctgagtggcctgggcctggtgggaaatagaccccgggtactcaggtgcttctctgaatcactggaaaggctgtcgaatgggagaaggaataaactccaacggcgcctgggcttgaactgagtgaaattaacaattaccgtgtagtgtttttgtaactgatcgttaatttaagggaaaaaattaaagaattagatgaaagttatagggaggtggatttgggttcattgtaagtagactttgccataaataaatgctgcctgggatcactgcataagctcttggtccacccaggtccgacgtgttggagtggggctcagcgaccctcagcctagctgctgccctggaggtggatttcagtctctgcgtgccggccggctcccagagttgcgagaggccggctccgcggtctcccagctacctcccggctgacttttcaccttccgctcccctttcctcctagtctcgaccctactacaccaccgtcccctcccaagtcccgggcagtgagaagatgcccggcatggggggcagccggagcctccctttagcagccagagtaggaagggggcttagtgagggagcccagacccaaacttcatccgcagctttcttcggcggaccttaccctctcctccttcagtggcattttggcatctattgtcgtcatatctgtctgctgccccacttaatctacaaatcgctcacgggtcggaggcaggacccgtgcgttttcagatgtactagctgggctgttctaactgcagggaaaaagcttacaaaacaagagttaattttaaaaacgtttcaaagaaagatgtgtttttaaaaataagttaataaaataacactcccttttccctcctggcagtgttttaaaattattgtttgaaacaaggtgtcagtttaagaatggtgtttataattaacttcatttaaacagtaatatttattaaattttaattgcagaactgtaagaaaacaaaaatggtttttaatcctaccacccacagattaacacttgttgaaataatgtcattgtttttaaactttcaattttttagctcagtgagagcatttttaattaactctctttcaaactgaacctagctgcctgtcaatatttgctcctaacaatgccagttagtaaacggactgattgtttctttcatttttattatgagacatttcaaacatatatttaaaacaaaaccagatagaataacataaacgtatcctgcttcattaactatcaaaactcagggctaatcttcttcccgtctgtaaatgagctgctttttgcatatggtacaacaaaaagaatgaggggaggtttgagcctggggaacctgccgtggcagcctgtccttccaggtgaagaccctgagatggagagatggtttggacagagcttcccaggtgggcaaacacgattttaaatacctgcctccctgctaacttactgtgtaaccctgggcaagtcacttaacctctctgagctctggtttcctcattgagaaaatagttgtttaatgattaaaggtacctcatatgagctcaaataatattaatccccatccctagtcccttccctttaaggtagtatgtcagattagtagcataagaagatccaaacctgtgtgtcctcttagtccagcgttcttcctcccttatgcagtttccgtcatcaacattgcctttctgttgccctcataacttatcatacggagccaggctatataattagctacttctctatccgcctcttggtacttaccaggcaagcttacctgtcatttccagctatcagctatttgtcaagcatcagtcacccccaacagcccccctgccatgcatttctactgttaatatctgtatctgtctccagagctctctaatctgtcccaccccgtagctgttttacatctagccatatacttctgtctgctctcattaaactgcctccccaaaactggctaatttatatttccgattttctattagttatatgttcttcctaacaataagaactatttacccatttgttcattatctttgtcatctattttaccttctgtgtttccaccattcatctcaaacttcatctccatagagctatttcgcaactgacaaacagtatattcatatgtctggtaatggttatctattattggctctggctttgtcttctctctgggtctgggcctcagtttctgtatctgtgagattgaatgacacaaattccagggttttttctagtgctgagtttctgtgactcctctacattctacttctctgtgtttctgtatactacctcctccacattctcagagctcaccacacaacccctgcctatcatgatatgcatcaaactttgttgttattacttaattatctgccatgtccaaacatcaatctgtagaccagcagtatgcgtctctcagggagatcttaaaatacagattcctgggtttcacccaggagattctcttaggaagtccaggatagggtgcaggaaaaagtttaaaaacagttatttgggtgatcatgattaataacaggcctgagcatcttagctctgggaggcagaggccaagcctgtctgtttcttacaggacccagctcagtgcccgggatggagtacatgctcaataaacatgtattgaattaatgagcacatttctctttgcccatacaaatacacactaactttatcagtcattccccttgctctctgctgtcattgctccctccctgtccctctccttctatctttcccttgtactttcacagctgattgttgatttagattatgcatataccagtttgtggataaaacttctcggagggttactcagatcagtgtgtgaatgagctcttaatccagatctcagaagtctgtgcactccccaagctttagccgggtgctaggaggtgggcaacctgggtgactctgtgtgtttagtgggagtggggtattcgtgctgggatggccagtgcctcaatctaggagatgagggaagagccctgggcaagggctagttctcccttcaggttctaatgacttgttcctcactgcttgggtgccgccctggagtatgaccaggaaggtaccagtctaagcttcagtcctggtggctggttgggcagacctgggcctgggtcattgcagaggctcaagtttaatgagtatgtgtaatgggtgtgtgcaacatgtgtctgcccatgtggggcaccaacgggctttatgtgattgatgcccaaaggtcagatgatagcataggtacacattagatgccattaggcagtcatatgacatggagtgcagcttgcatgcttttgtgtgtgttcgtgtgtgtgtcgggggcaggggtaagttagttttagggggagtgagagaaagcacctggttgctccaggctgatcaactggtcagtgtttccagctactccttctgctctgaacagatcagcaggtgtttcttgaccttgcctgggttagagtttagctgagcggtgaaggcaaagggtacagaaacgtggcctgtggctttgaagatttcttactgagtgatgaaggctaagtgcaaagcttgcacatttgtgaaacatgcacaggaagaatgactagggtcccctttgaggtcacagctgtgggctgaggggtgtcaggatagaaacgcttgagaagatggctccaggaggcctcagacctggaagacttggggggatgcctaggatcctaggttggagggaaagaagggcagggtttgaggcaggcagatgaagatagagccaccatcttggagcccaagggcagggagatcttgggaggcaggagttacggtcacctgcctatggctttttcccctcagaggcatggaaaggaggatttggagggtcctttcctgctctggaatgttctggccttagagggatggataagagggggatatccaagtgacctgaattttagggaaaaatcaagagacatttgttcctagctcacggtgtgtccacatctcttctctaagtcttggcttttcttcaagaacttctgcatctcatgttccaggagtcctgtgtgggaggatgagggggagataaaggagattagagtggttctgtgaggagctgggaccaacatgtcctgaggtgaatcttatgatgtctccctgagagagacagaggaagggtccaggctgggctgaaagaggaggagacagggaggcttagggagatcatggttatggttggtggggagctggaggtgacctcagcttactgaggtgaaggttgaacttagcatggcattgattgggcttgaccttgagagtgggaacagcccacatgatcaaatgataggaaatgggtccccagggaagagagaaagctgaggggtgacttgactgatatctccaggctcctgtccattctgggatatttgaaatctttgaagacaggacacgtattcacctgaaagtgtgcaggggcctggagccacagacttttccatttgcaggagtggtgaaaaagaagggatccagacctcgttcattcagaatagcagattattccaaagtaaagtctgattagttctgaaatatcggctggagccatagtttgcttgtttgttagttcatttttccctttgttcttgcatgcatgtcttcatttattaatgcatacattgatcagtcctctagcaaactgatacattcattcatccatagcagtttcaccttcttcattctgcctgactcaagccaacccttcttctgcccagcagtaggtgtccctcctccaacttcccctaaaagtggccaatccaatttaccatgtggaatattaaaaactggccctcttgcaaaagtgtccacaaaactaagaaaaagatccagtttctccatcattgagcacttctcaaagcctttgctgattagaattctacccctcttctgttcattttctcctgttttccaggtctggcccaggtacctcttgcctagagcataggcttgtccagccagatgactatacatggaacatgtcctctgggcagggcactgggactaacataacagtttggctctccagtctcatagtctggtgaggaggcagacgtaaataaataaattagtgcacagtgggggtcactgttactgagactgggaagaggtactaaggaactacaggcaggtgatggggcaggaccattaaggaacatcaggacagggtcttgaaggctaaggagagtattccagggttggtaagtcaggagaatggagacttttggaaggatgtggcctctgagaaactgagatgttcacttcacagtgaaatgaggacttgggagaccacaagggacctcttgctacagcagagaggtcagagtgggcaaggggtcctccagctaacattccaactgtacctcggggcttagagagaggtgagtagtgtgtttgtgttggggatggggaggcatgtgcaggacagatccagcctccaagccataccatatgacccagctcctttccagggcctgttttctctagggaaggggctctgaaggatccagagttgcctggctgggttggagaggtcatgaaatgtcactctcatctcctaatacactcagagcccagttccttttctttttccaagtaaaaaataactaccattatcaataatctattaaggaaaattcagaaaagtagaaagaagaaagaaacatcacccacactttaggtatatttccttctagtcttttttccccgtgtgtagattttgtttttctatggttgtgatcacactgtgccagccttgtgcatcctggcgtttccattaatgctatgaagtcataagcactaccctgttattgcagtctttgtaaacagcatctggacactcagcccaaggctgttctccggaagatggccaggctgcacagggagagggtttatgtccctgcctctagagagatgcctacttgaccccagtatttttcatggagaaaatattcagaatcacctttcacttgggtgccctaggaagctgcctctggcctatcctgtgcctgaagtcgccatccaaagctttccttctttgagccagtgttgctagtcaagggcagcatgctgggcccgtcccactacaggccaatgtgaccgtcagtctccttcctgaaggacacttggaaatgcatgtggaaagaggaaggtacagaaaagggcccccggtccctggtactgcccgcatcacctgacagtcaccttcggccagcccacttgggcttctcaggaatgacaccccggccctgcatctggccctgagtcacgcacaggaggcagggtgagctcacccgcccactgactggcacagtcatagcaggctccagggtggggggcaggggccaggctgctgccaaatggttgtgctgagaaccacccagggtccaggtggccctgcgcccaaagataggtgggcttggagtccagcagcctgtgcccagagcctctgccatcctccacggccggcctaggtgagatgtgcaggctatgggcttggaaatgaggggagaatccccttgccctcactccatccatcgaggccgggcaccaacccttcctgggccagctttccagcccctggctggctgctctgcaggcactgaatgccagctgcccccatccccatgccagtgctctaaaatcagtgctctcaaacaagggcagatggcgcagtggaagttctggcaagaggggactgtgaggggaagtcctggggtaggtgggacagagaggactgcctgggaagggtgtaggggcagcacctcctgggcatgaaaccatctgcagggcacaggggccaggcctgcctctgcatgcactgcttggccttgtggctaaggcctgtgctttacccagttctctgggagcaggagcagtctttctgaggcctgccctcagccctgcccagggttcaaggatctctcctcagcatcattgctgctgccaaaaccaagaggctacccaccattcctcacccgcaactctgccacgcagcaccgtctgcacagctgcagttggccacatccacttgcttttaaatgtgctgtcatttcctggaaaccatccaggccttgtagcctgccctctgcacctcctccccaaggggggcctctggagcaagaatccaagaggtgccctggcagctgcaagtgtccccagaacatttcctctatgcatgaaggactgaagcccagagggggaagggacttagctgagaatcagtacccaggatcctcctgccaacgctgaagatggtttgggtctggcctgactctgcaaagccaagtaaagaaccacggagtcagggagagttgacagatgaaggctttctccacagcccacaagcactaagtccagtccaggagccaggatgagcctcccagattatgcatgagaggacattaagggctgtgtcctggacactgaacagatgctggaggaggagggaaaagaggcttcctggaggagatggcttagaaccatagacctgccctctgcctcatgcctcctccatcatggaggatggttgtccagtttctgtttgaaccccaccccataccttgccagggctctcactgccagacacagaatagggggctccctgggttcaaagtagagctcacttctgtcccctgggcttctcctgactgttccttgtgtgacctgttcccacatctggatgggctgcaggagccagtgctgtggggacagaaggtctggagctgcccgtgaagggcagaatgctgccctcagacccgcttcctccctgtccttgtctgtccaaggagaatgaggtctcactggtggatttcggactaccctgaggagctggcacctgagggacaaggccccccacctgcccagctccagcctctgatgaggggtgggagagagctacatgaggttgctaagaaagcctcccctgaaggagaccacacagtgtgtgaggttggagtctctagcagcgggttctgtgcccccagggatagtctggctgtccaggcactgctcttgatataaacaccacctcctagttatgaaaccatgcccattctgcctctctgtatggaaaagagcatggggctggcccgtggggtggtgtccactttaggccctgtgggagatcatgggaacccacgcagtgggtcataggctctctcatttactactcacatccactctgtgaagaagcgattatgatctctcctctagaaactcgtagagtcccatgtctgccggcttccagagcctgcactcctccaccttggcttggctttgctggggctagaggagctaggatgcacagcagctctgtgaccctttgtttgagaggaacaggaaaaccacccttctctctggcccactgtgtcctcttcctgccctgccatccccttctgtgaatgttagacccatgggagcagctggtcagaggggaccccggcctggggcccctaaccctatgtagcctcagtcttcccatcaggctctcagctcagcctgagtgttgaggccccagtggctgctctgggggcctcctgagtttctcatctgtgcccctccctccctggcccaggtgaaggtgtggttccagaaccggaggacaaagtacaaacggcagaagctggaggaggaagggcctgagtccgagcagaagaagaagggctcccatcacatcaaccggtggcgcattgccacgaagcaggccaatggggaggacatcgatgtcacctccaatgactagggtgggcaaccacaaacccacgagggcagagtgctgcttgctgctggccaggcccctgcgtgggcccaagctggactctggccactccctggccaggctttggggaggcctggagtcatggccccacagggcttgaagcccggggccgccattgacagagggacaagcaatgggctggctgaggcctgggaccacttggccttctcctcggagagcctgcctgcctgggcgggcccgcccgccaccgcagcctcccagctgctctccgtgtctccaatctcccttttgttttgatgcatttctgttttaatttattttccaggcaccactgtagtttagtgatccccagtgtcccccttccctatgggaataataaaagtctctctcttaatgacacgggcatccagctccagccccagagcctggggtggtagattccggctctgagggccagtgggggctggtagagcaaacgcgttcagggcctgggagcctggggtggggtactggtggagggggtcaagggtaattcattaactcctctcttttgttgggggaccctggtctctacctccagctccacagcaggagaaacaggctagacatagggaagggccatcctgtatcttgagggaggacaggcccaggtctttcttaacgtattgagaggtgggaatcaggcccaggtagttcaatgggagagggagagtgcttccctctgcctagagactctggtggcttctccagttgaggagaaaccagaggaaaggggaggattggggtctgggggagggaacaccattcacaaaggctgacggttccagtccgaagtcgtgggcccaccaggatgctcacctgtccttggagaaccgctgggcaggttgagactgcagagacagggcttaaggctgagcctgcaaccagtccccagtgactcagggcctcctcagcccaagaaagagcaacgtgccagggcccgctgagctcttgtgttcacctgcccttctgtttgtcccacttgtcaggatgaaggtttcctgacaagcaaatctgcattcctaagtctttcccttacgacatccagacccctctctttcttcttcacctcccatgtgctcatgaaacctctgctctttggcctccatgccaccattctgccggtgctaatgacagtcaccaaccacagtcactggccacccccttgtggccaaactcaaccacttcctgttgggttcacctgctccctgatctgttggctatgccctcctggattctcccaccccgctctgccttcatttcggtagctctgactcctccttcagcctgagttcattcagtgtgatccatgccttgtcacctctggccacccccaggtcagtccttgctctccctgactcctcattatgtcctttgccttgtggggatcacatccacttccaggacttctctttggctccctggcctgtgtctttagctgacctctgctgagctgcagacccgtcaagccagctgcctgctccaccccctgcccctcagcacctcaaagcccatacatccacagccggacgcacctacccatctgtgcttctccaggatcacccacctcgacaaacagcattagacatgtacacagtttcccaagctacaggaaatctgggaatcttcctcaagcttcctctcctcttccccagccccatccattcccatctagtgggttgagtctagactggcttcccaaccacacctccctaatgcagcaccccctacccccctgcccagctccctctgccaccggcctggcctgggccctgctcctctagggaggtttctgtgaatgtcaaggatgaggtccacttcaaaggaggccctccatgttgcagctaggtttctcttccttgcacccaaacagggcagactcacccccttctgagcccctttgccccatcttcttgccttgctcccggtaccctttgcttcagcatccccatccctgtccctgagtgagccacaggttttccctgtgctgtgccttcgctcatgctgttcttcccacctggaatgtcgggtgcttgatcaatgtggaactcactggaaagatgtcagagacccagccttgctgtctgggccacatgcagggatccaagcacacaaggtccttctgctgggagcacagacccaggtcccactcgcactctcagcgtctctctcccacctctgcccacctcacttgtgtccagtcagtgctagaaaccaaagggctttgtcccatcccaacaccccctctccctccatcagtcaggaatgcattctgcacatcttgaaagtcctaacatggataagtccagattaacccacatggcgaccctcactgccaagcaggtgggatcacttctgggagcacacatgcccaggtgtggaaggaaggtgggaggaagagtcatccttttggccccagtgggggacagagaaaggggtgagctgttcctctcaagatcctgcctcacttggtagggggagggggtccaggaagatcacagcagagcaccccctgtcatccgaataaagggctggaagggacccaaggaaacctgccagtctcccgaggccaggcctgcggggggcggggcggggagtccctgccgcactcccatccaccccccatgttgtgcctctccctgcagacggtaaatattggtgttgtgacttcattaataaaggcttctgtgagcctgaaaaa

SEQ ID NO: 50 - DNA, 30 bp, Artificial Sequence
  primer1 (EMX1)
gggcttctcctgactgttccttgtgtgacc

SEQ ID NO: 51 - DNA, 30 bp, Artificial Sequence
  primer2 (EMX1)
caggatggcccttccctatgtctagcctgt

SEQ ID NO: 52 - protein, 7 aa, Artificial Sequence
  NLS (protein)
PKKKRKV

SEQ ID NO: 53 - DNA, 21 bp, Artificial Sequence
  NLS (nucleotide)
cccaagaagaagcggaaggtg

SEQ ID NO: 54 - protein, 19 aa, Artificial Sequence
  BPNLS (protein)
KRTADGSEFESPKKKRKVE

SEQ ID NO: 55 - DNA, 57 bp, Artificial Sequence
  BPNLS (nucleotide)
aagcggactgctgatggcagtgaatttgagtccccaaagaagaagagaaaggtggaa

SEQ ID NO: 56 - DNA, 44 bp, Artificial Sequence
  BPNLS insert upper
agatcttaatacgactcactatagggagagccgccaccatggcc

SEQ ID NO: 57 - DNA, 13 bp, Artificial Sequence
  BPNLS insert lower
taatatcctcgag

SEQ ID NO: 58 - protein, 22 aa, Artificial Sequence
  2A (protein)
GSGATNFSLLKQAGDVEENPGP

SEQ ID NO: 59 - DNA, 66 bp, Artificial Sequence
  2A (nucleotide Cse1-Cse2)
ggaagcggagcaaccaacttcagcctgctgaagcaggccggcgatgtggaggagaatccaggcccc

SEQ ID NO: 60 - DNA, 66 bp, Artificial Sequence
  2A(nucleotide Cse2-Cas7)
ggctccggcgccaccaatttttctctgctgaagcaggcaggcgatgtggaggagaacccaggacct

SEQ ID NO: 61 - DNA, 66 bp, Artificial Sequence
  2A(nucleotide Cas7-Cas5)
ggatctggagccaccaatttcagcctgctgaagcaagcaggcgacgtggaagaaaacccaggacca

SEQ ID NO: 62 - DNA, 66 bp, Artificial Sequence
  2A(nucleotide Cas5-Cas6)
ggatctggggctactaatttttctctgctgaagcaagccggcgacgtggaagagaatccaggaccg

SEQ ID NO: 63 - DNA, 176 bp, Artificial Sequence
  pre-crRNA(LRSR)
tggatgtgttgtttgtgtgatactataaagttggtagattgtgactggcttaaaaaatcattaattaataataggttatgtttagagtgttccccgcgccagcggggataaaccgcaggccaatggggaggacatcgatgtcacctcgtgttccccgcgccagcggggataaaccg

SEQ ID NO: 64 - DNA, 90 bp, Artificial Sequence
  pre-crRNA(RSR)
gtgttccccgcgccagcggggataaaccgcaggccaatggggaggacatcgatgtcacctcgtgttccccgcgccagcggggataaaccg

SEQ ID NO: 65 - DNA, 61 bp, Artificial Sequence
  mature crRNA
ataaaccgcaggccaatggggaggacatcgatgtcacctcgtgttccccgcgccagcgggg